European Patent Application EP 4 166 572 A1, published April 19, 2023. Title: ANTI-PD-1 ANTIBODIES AND METHODS OF USE THEREOF. Applicant: Rinat Neuroscience Corp. The sequence listing filed with the application follows.

SEQUENCE LISTING (51 sequences)

SEQ ID NO: 1 - protein, 288 aa, Homo sapiens
MQIPQAPWPVVWAVLQLGWRPGWFLDSPDRPWNPPTFSPALLVVTEGDNATFTCSFSNTSESFVLNWYRMSPSNQTDKLAAFPEDRSQPGQDCRFRVTQLPNGRDFHMSVVRARRNDSGTYLCGAISLAPKAQIKESLRAELRVTERRAEVPTAHPSPSPRPAGQFQTLVVGVVGGLLGSLVLLVWVLAVICSRAARGTIGARRTGQPLKEDPSAVPVFSVDYGELDFQWREKTPEPPVPCVPEQTEYATIVFPSGMGTSSPARRGSADGPRSAQPLRPEDGHCSWPL

SEQ ID NO: 2 - protein, 113 aa, synthetic construct
  REGION 1..113: note = humanized antibody sequence
DIVMTQSPDSLAVSLGERATINCKSSQSLWDSGNQKNFLTWYQQKPGQPPKLLIYWTSTRESGVPDRFSGSGSGTDFTLTISSLQAEDVAVYYCQNDYFYPLTFGGGTKVEIK

SEQ ID NO: 3 - protein, 117 aa, synthetic construct
  REGION 1..117: note = humanized antibody sequence
QVQLVQSGAEVKKPGASVKVSCKASGYTFTSYWINWVRQAPGQGLEWMGNIYPGSSLTNYNEKFKNRVTMTRDTSTSTVYMELSSLRSEDTAVYYCARLLTGTFAYWGQGTLVTVSS

SEQ ID NO: 4 - protein, 117 aa, synthetic construct
  REGION 1..117: note = humanized antibody sequence
QVQLVQSGAEVKKPGASVKVSCKASGYTFTSYWINWVRQAPGQGLEWMGNIYPGSSLTNYNEKFKNRVTMTRDTSTSTVYMELSSLRSEDTAVYYCARLSTGTFAYWGQGTLVTVSS

SEQ ID NO: 5 - protein, 117 aa, synthetic construct
  REGION 1..117: note = humanized antibody sequence
QVQLVQSGAEVKKPGASVKVSCKASGYTFTSYWINWVRQAPGQGLEWMGNIYPGSSITNYNEKFKNRVTMTRDTSTSTVYMELSSLRSEDTAVYYCARLTTGTFAYWGQGTLVTVSS

SEQ ID NO: 6 - protein, 117 aa, synthetic construct
  REGION 1..117: note = humanized antibody sequence
QVQLVQSGAEVKKPGASVKVSCKASGYTFTSYWINWVRQAPGQGLEWMGNIWPGSSLTNYNEKFKNRVTMTRDTSTSTVYMELSSLRSEDTAVYYCARLLTGTFAYWGQGTLVTVSS

SEQ ID NO: 7 - protein, 113 aa, synthetic construct
  REGION 1..113: note = humanized antibody sequence
DIVMTQSPDSLAVSLGERATINCKSSQSLWDSGNQKNFLTWYQQKPGQPPKLLIYWTSYRESGVPDRFSGSGSGTDFTLTISSLQAEDVAVYYCQNDYFYPLTFGGGTKVEIK

SEQ ID NO: 8 - protein, 113 aa, synthetic construct
  REGION 1..113: note = humanized antibody sequence
DIVMTQSPDSLAVSLGERATINCKSSQSLWDSGNQKNFLTWYQQKPGQPPKLLIYWTSYRESGVPDRFSGSGSGTDFTLTISSLQAEDVAVYYCQNDYFYPHTFGGGTKVEIK

SEQ ID NO: 9 - protein, 113 aa, synthetic construct
  REGION 1..113: note = humanized antibody sequence
DIVMTQSPDSLAVSLGERATINCKSSQSLWDSTNQKNFLTWYQQKPGQPPKLLIYWTSTRESGVPDRFSGSGSGTDFTLTISSLQAEDVAVYYCQNDYFYPLTFGGGTKVEIK

SEQ ID NO: 10 - protein, 17 aa, synthetic construct
  REGION 1..17: note = humanized antibody sequence
KSSQSLWDSGNQKNFLT

SEQ ID NO: 11 - protein, 7 aa, synthetic construct
  REGION 1..7: note = humanized antibody sequence
WTSTRES

SEQ ID NO: 12 - protein, 9 aa, synthetic construct
  REGION 1..9: note = humanized antibody sequence
QNDYFYPLT

SEQ ID NO: 13 - protein, 10 aa, synthetic construct
  REGION 1..10: note = humanized antibody sequence
GYTFTSYWIN

SEQ ID NO: 14 - protein, 7 aa, synthetic construct
  REGION 1..7: note = humanized antibody sequence
GYTFTSY

SEQ ID NO: 15 - protein, 5 aa, synthetic construct
  REGION 1..5: note = humanized antibody sequence
SYWIN

SEQ ID NO: 16 - protein, 6 aa, synthetic construct
  REGION 1..6: note = humanized antibody sequence
YPGSSL

SEQ ID NO: 17 - protein, 17 aa, synthetic construct
  REGION 1..17: note = humanized antibody sequence
NIYPGSSLTNYNEKFKN

SEQ ID NO: 18 - protein, 8 aa, synthetic construct
  REGION 1..8: note = humanized antibody sequence
LLTGTFAY

SEQ ID NO: 19 - protein, 15 aa, synthetic construct
  REGION 1..15: note = Synthetic linker
GGGGSGGGGSGGGGS

SEQ ID NO: 20 - protein, 7 aa, synthetic construct
  REGION 1..7: note = humanized antibody sequence
WTSYRES

SEQ ID NO: 21 - protein, 9 aa, synthetic construct
  REGION 1..9: note = humanized antibody sequence
QNDYFYPHT

SEQ ID NO: 22 - protein, 17 aa, synthetic construct
  REGION 1..17: note = humanized antibody sequence
KSSQSLWDSTNQKNFLT

SEQ ID NO: 23 - protein, 8 aa, synthetic construct
  REGION 1..8: note = humanized antibody sequence
LSTGTFAY

SEQ ID NO: 24 - protein, 6 aa, synthetic construct
  REGION 1..6: note = humanized antibody sequence
YPGSSI

SEQ ID NO: 25 - protein, 17 aa, synthetic construct
  REGION 1..17: note = humanized antibody sequence
NIYPGSSITNYNEKFKN

SEQ ID NO: 26 - protein, 8 aa, synthetic construct
  REGION 1..8: note = humanized antibody sequence
LTTGTFAY

SEQ ID NO: 27 - protein, 6 aa, synthetic construct
  REGION 1..6: note = humanized antibody sequence
WPGSSL

SEQ ID NO: 28 - protein, 17 aa, synthetic construct
  REGION 1..17: note = humanized antibody sequence
NIWPGSSLTNYNEKFKN

SEQ ID NO: 29 - protein, 444 aa, synthetic construct
  REGION 1..444: note = humanized antibody sequence
QVQLVQSGAEVKKPGASVKVSCKASGYTFTSYWINWVRQAPGQGLEWMGNIYPGSSLTNYNEKFKNRVTMTRDTSTSTVYMELSSLRSEDTAVYYCARLSTGTFAYWGQGTLVTVSSASTKGPSVFPLAPCSRSTSESTAALGCLVKDYFPEPVTVSWNSGALTSGVHTFPAVLQSSGLYSLSSVVTVPSSSLGTKTYTCNVDHKPSNTKVDKRVESKYGPPCPPCPAPEFLGGPSVFLFPPKPKDTLMISRTPEVTCVVVDVSQEDPEVQFNWYVDGVEVHNAKTKPREEQFNSTYRVVSVLTVLHQDWLNGKEYKCKVSNKGLPSSIEKTISKAKGQPREPQVYTLPPSQEEMTKNQVSLTCLVKGFYPSDIAVEWESNGQPENNYKTTPPVLDSDGSFFLYSRLTVDKSRWQEGNVFSCSVMHEALHNHYTQKSLSLSLGK

SEQ ID NO: 30 - protein, 17 aa, synthetic construct
  REGION 1..17: note = humanized antibody sequence
KSSQSLLDSGNQKNFLT

SEQ ID NO: 31 - protein, 9 aa, synthetic construct
  REGION 1..9: note = humanized antibody sequence
QNDYSYPLT

SEQ ID NO: 32 - protein, 17 aa, synthetic construct
  REGION 1..17: note = humanized antibody sequence
  VARIANT 7: note = Xaa is Trp or Leu
  VARIANT 10: note = Xaa is Gly or Thr
KSSQSLXDSXNQKNFLT

SEQ ID NO: 33 - protein, 7 aa, synthetic construct
  REGION 1..7: note = humanized antibody sequence
  VARIANT 4: note = Xaa is Thr or Tyr
WTSXRES

SEQ ID NO: 34 - protein, 9 aa, synthetic construct
  REGION 1..9: note = humanized antibody sequence
  VARIANT 5: note = Xaa is Phe or Ser
  VARIANT 8: note = Xaa is Leu or His
QNDYXYPXT

SEQ ID NO: 35 - protein, 17 aa, synthetic construct
  REGION 1..17: note = humanized antibody sequence
NIYPGSSSTNYNEKFKN

SEQ ID NO: 36 - protein, 17 aa, synthetic construct
  REGION 1..17: note = humanized antibody sequence
  VARIANT 3: note = Xaa is Tyr or Trp
  VARIANT 8: note = Xaa is Leu, Ile, or Ser
NIXPGSSXTNYNEKFKN

SEQ ID NO: 37 - protein, 8 aa, synthetic construct
  REGION 1..8: note = humanized antibody sequence
  VARIANT 2: note = Xaa is Leu or Ser
LXTGTFAY

SEQ ID NO: 38 - protein, 443 aa, synthetic construct
  REGION 1..443: note = humanized antibody sequence
QVQLVQSGAEVKKPGASVKVSCKASGYTFTSYWINWVRQAPGQGLEWMGNIYPGSSLTNYNEKFKNRVTMTRDTSTSTVYMELSSLRSEDTAVYYCARLSTGTFAYWGQGTLVTVSSASTKGPSVFPLAPCSRSTSESTAALGCLVKDYFPEPVTVSWNSGALTSGVHTFPAVLQSSGLYSLSSVVTVPSSSLGTKTYTCNVDHKPSNTKVDKRVESKYGPPCPPCPAPEFLGGPSVFLFPPKPKDTLMISRTPEVTCVVVDVSQEDPEVQFNWYVDGVEVHNAKTKPREEQFNSTYRVVSVLTVLHQDWLNGKEYKCKVSNKGLPSSIEKTISKAKGQPREPQVYTLPPSQEEMTKNQVSLTCLVKGFYPSDIAVEWESNGQPENNYKTTPPVLDSDGSFFLYSRLTVDKSRWQEGNVFSCSVMHEALHNHYTQKSLSLSLG

SEQ ID NO: 39 - protein, 221 aa, synthetic construct
  REGION 1..221: note = humanized antibody sequence
DIVMTQSPDSLAVSLGERATINCKSSQSLWDSGNQKNFLTWYQQKPGQPPKLLIYWTSYRESGVPDRFSGSGSGTDFTLTISSLQAEDVAVYYCQNDYFYPHTFGGGTKVEIKRGTVAAPSVFIFPPSDEQLKSGTASVVCLLNNFYPREAKVQWKVDNALQSGNSQESVTEQDSKDSTYSLSSTLTLSKADYEKHKVYACEVTHQGLSSPVTKSFNRGEC

SEQ ID NO: 40 - DNA, 351 bp, synthetic construct
  misc_feature 1..351: note = mAb7 heavy chain variable region DNA sequence
  source 1..351: mol_type = other DNA
caggtgcagctggtgcagagcggcgccgaagtgaagaaaccaggagccagcgtgaaagtgagttgtaaggcatccggctatacctttacctcttactggatcaattgggtgaggcaggcacctggccagggcctggaatggatgggaaatatctatcccggctctagcttgactaactacaatgaaaagtttaagaatcgcgtgaccatgacccgggacactagcacctccaccgtgtacatggagctgtcctccctgcggagcgaggacaccgccgtctactattgtgcccgcctgagtaccgggacctttgcctactggggacagggtacactggtcaccgtctcctca

SEQ ID NO: 41 - DNA, 339 bp, synthetic construct
  misc_feature 1..339: note = mAb7 light chain variable region DNA sequence
  source 1..339: mol_type = other DNA
gacatcgtgatgactcagtctcccgatagcctggcagtcagcctgggagagcgggccaccataaactgcaaaagctcgcagtcgctgtgggacagtggtaatcagaagaatttcctgacctggtaccagcagaagcctggccagccacccaagctgctgatctactggacctcatatcgggagtccggggtgcccgacagattctctggaagtggcagcggtacggacttcacactgaccatatccagtctgcaagctgaggacgtggctgtttattactgccagaacgactacttttatcctcacactttcggaggcggtaccaaggtcgagatcaaa

SEQ ID NO: 42 - protein, 750 aa, Homo sapiens
MWNLLHETDSAVATARRPRWLCAGALVLAGGFFLLGFLFGWFIKSSNEATNITPKHNMKAFLDELKAENIKKFLYNFTQIPHLAGTEQNFQLAKQIQSQWKEFGLDSVELAHYDVLLSYPNKTHPNYISIINEDGNEIFNTSLFEPPPPGYENVSDIVPPFSAFSPQGMPEGDLVYVNYARTEDFFKLERDMKINCSGKIVIARYGKVFRGNKVKNAQLAGAKGVILYSDPADYFAPGVKSYPDGWNLPGGGVQRGNILNLNGAGDPLTPGYPANEYAYRRGIAEAVGLPSIPVHPIGYYDAQKLLEKMGGSAPPDSSWRGSLKVPYNVGPGFTGNFSTQKVKMHIHSTNEVTRIYNVIGTLRGAVEPDRYVILGGHRDSWVFGGIDPQSGAAVVHEIVRSFGTLKKEGWRPRRTILFASWDAEEFGLLGSTEWAEENSRLLQERGVAYINADSSIEGNYTLRVDCTPLMYSLVHNLTKELKSPDEGFEGKSLYESWTKKSPSPEFSGMPRISKLGSGNDFEVFFQRLGIASGRARYTKNWETNKFSGYPLYHSVYETYELVEKFYDPMFKYHLTVAQVRGGMVFELANSIVLPFDCRDYAVVLRKYADKIYSISMKHPQEMKTYSVSFDSLFSAVKNFTEIASKFSERLQDFDKSNPIVLRMMNDQLMFLERAFIDPLGLPDRPFYRHVIYAPSSHNKYAGESFPGIYDALFDIESKVDPSKAWGEVKRQIYVAAFTVQAAAETLSEVA

SEQ ID NO: 43 - DNA, 2217 bp, synthetic construct
  misc_feature 1..2217: note = Synthetic Construct
  source 1..2217: mol_type = other DNA
atggctagcgccagacgccccagatggctgtgtgctggcgctctggtgctggctggcggcttcttcctgctgggcttcctgttcggctggttcatcaagtcctccaacgaggccaccaacatcacccccaagcacaacatgaaggcctttctggacgagctgaaggccgagaatatcaagaagttcctgtacaacttcacccagatcccccacctggccggcaccgagcagaacttccagctggccaagcagatccagtcccagtggaaagagttcggcctggactccgtggaactggcccactacgacgtgctgctgtcctaccccaacaagacccaccccaactacatctccatcatcaacgaggacggcaacgaaatcttcaacacctccctgttcgagcccccacccccaggctacgagaacgtgtccgacatcgtgcccccattctccgccttcagtccacaaggcatgcccgagggcgacctggtgtacgtgaactacgccaggaccgaggacttcttcaagctggaacgcgacatgaagatcaactgctccggcaagatcgtgatcgccagatacggcaaggtgttcaggggcaacaaagtgaagaacgcccagctggctggggccaagggcgtgatcctgtactccgaccccgccgactacttcgccccaggcgtgaagtcctaccccgacggatggaacctgccaggcggcggagtgcagaggggcaacatcctgaacctgaacggcgctggcgaccccctgaccccaggatacccagccaacgagtacgcctacagaagaggaatcgccgaggccgtgggcctgccctctatcccagtgcaccccatcggctactacgacgcccagaaactgctggaaaagatgggcggctccgccccacccgactcctcttggagaggctccctgaaggtgccctacaacgtgggcccaggcttcaccggcaacttctccacccagaaagtgaagatgcacatccactccaccaacgaagtgaccaggatctacaacgtgatcggcaccctgagaggcgccgtggaacccgacagatacgtgatcctgggcggccacagggacagctgggtgttcggcggcatcgacccacagtctggcgccgctgtggtgcacgagatcgtgcggtccttcggaaccctgaagaaagagggatggcgccccagaaggaccatcctgttcgccagctgggacgccgaggaattcggcctgctgggatccaccgagtgggccgaggaaaactccaggctgctgcaggaacgcggcgtcgcctacatcaacgccgactcctccatcgagggcaactacaccctgagggtggactgcacccccctgatgtactccctggtgcacaacctgaccaaagagctgaagtcccccgacgagggcttcgagggcaagtccctgtacgagtcctggaccaagaagtccccatcccccgagttctccggcatgcccaggatctccaagctgggctccggcaacgacttcgaggtgttcttccagaggctgggaatcgcctccggcagggccagatacaccaagaactgggagacaaacaagttctccggataccccctgtaccactccgtgtacgaaacctacgagctggtggaaaagttctacgaccccatgttcaagtaccacctgaccgtggcccaagtccgcggaggcatggtgttcgagctggccaactccatcgtgctgcccttcgactgcagagactacgccgtggtgctgaggaagtacgccgacaaaatctactccatctccatgaagcacccccaggaaatgaagacctactccgtgtccttcgactccctgttctccgccgtgaagaatttcaccgagatcgcctccaagttcagcgagaggctgcaggacttcgacaagtccaacccaatcgtgctgaggatgatgaacgaccagctgatgttcctggaaagggccttcatcgaccccctgggcctgccagacagacccttctacaggcacgtgatctacgccccatcctcccacaacaaatacgccggcgagtccttccccggcatctacgatgccctgttcgacatcgagtccaaggtggacccctccaaggcctggggcgaagtgaagaggcaaatctacgtggccgccttcacagtgcaagccgctgccgaaaccctgtccgaggtggcc

SEQ ID NO: 44 - DNA, 33562 bp, synthetic construct
  misc_feature 1..33562: note = Synthetic Construct
  source 1..33562: mol_type = other DNA
ccatcttcaataatatacctcaaactttttgtgcgcgttaatatgcaaatgaggcgtttgaatttggggaggaagggcggtgattggtcgagggatgagcgaccgttaggggcggggcgagtgacgttttgatgacgtggttgcgaggaggagccagtttgcaagttctcgtgggaaaagtgacgtcaaacgaggtgtggtttgaacacggaaatactcaattttcccgcgctctctgacaggaaatgaggtgtttctgggcggatgcaagtgaaaacgggccattttcgcgcgaaaactgaatgaggaagtgaaaatctgagtaatttcgcgtttatggcagggaggagtatttgccgagggccgagtagactttgaccgattacgtgggggtttcgattaccgtgtttttcacctaaatttccgcgtacggtgtcaaagtccggtgtttttactactgtaatagtaatcaattacggggtcattagttcatagcccatatatggagttccgcgttacataacttacggtaaatggcccgcctggctgaccgcccaacgacccccgcccattgacgtcaataatgacgtatgttcccatagtaacgccaatagggactttccattgacgtcaatgggtggagtatttacggtaaactgcccacttggcagtacatcaagtgtatcatatgccaagtacgccccctattgacgtcaatgacggtaaatggcccgcctggcattatgcccagtacatgaccttatgggactttcctacttggcagtacatctacgtattagtcatcgctattaccatggtgatgcggttttggcagtacatcaatgggcgtggatagcggtttgactcacggggatttccaagtctccaccccattgacgtcaatgggagtttgttttggcaccaaaatcaacgggactttccaaaatgtcgtaacaactccgccccattgacgcaaatgggcggtaggcgtgtacggtgggaggtctatataagcagagctgtccctatcagtgatagagatctccctatcagtgatagagagtttagtgaaccgtcagatccgctagggtaccgcgatcaccatggctagcgccagacgccccagatggctgtgtgctggcgctctggtgctggctggcggcttcttcctgctgggcttcctgttcggctggttcatcaagtcctccaacgaggccaccaacatcacccccaagcacaacatgaaggcctttctggacgagctgaaggccgagaatatcaagaagttcctgtacaacttcacccagatcccccacctggccggcaccgagcagaacttccagctggccaagcagatccagtcccagtggaaagagttcggcctggactccgtggaactggcccactacgacgtgctgctgtcctaccccaacaagacccaccccaactacatctccatcatcaacgaggacggcaacgaaatcttcaacacctccctgttcgagcccccacccccaggctacgagaacgtgtccgacatcgtgcccccattctccgccttcagtccacaaggcatgcccgagggcgacctggtgtacgtgaactacgccaggaccgaggacttcttcaagctggaacgcgacatgaagatcaactgctccggcaagatcgtgatcgccagatacggcaaggtgttcaggggcaacaaagtgaagaacgcccagctggctggggccaagggcgtgatcctgtactccgaccccgccgactacttcgccccaggcgtgaagtcctaccccgacggatggaacctgccaggcggcggagtgcagaggggcaacatcctgaacctgaacggcgctggcgaccccctgaccccaggatacccagccaacgagtacgcctacagaagaggaatcgccgaggccgtgggcctgccctctatcccagtgcaccccatcggctactacgacgcccagaaactgctggaaaagatgggcggctccgccccacccgactcctcttggagaggctccctgaaggtgccctacaacgtgggcccaggcttcaccggcaacttctccacccagaaagtgaagatgcacatccactccaccaacgaagtgaccaggatctacaacgtgatcggcaccctgagaggcgccgtggaacccgacagatacgtgatcctgggcggccacagggacagctgggtgttcggcggcatcgacccacagtctggcgccgctgtggtgcacgagatcgtgcggtccttcggaaccctgaagaaagagggatggcgccccagaaggaccatcctgttcgccagctgggacgccgaggaattcggcctgctgggatccaccgagtgggccgaggaaaactccaggctgctgcaggaacgcggcgtcgcctacatcaacgccgactcctccatcgagggcaactacaccctgagggtggactgcacccccctgatgtactccctggtgcacaacctgaccaaagagctgaagtcccccgacgagggcttcgagggcaagtccctgtacgagtcctggaccaagaagtccccatcccccgagttctccggcatgcccaggatctccaagctgggctccggcaacgacttcgaggtgttcttccagaggctgggaatcgcctccggcagggccagatacaccaagaactgggagacaaacaagttctccggataccccctgtaccactccgtgtacgaaacctacgagctggtggaaaagttctacgaccccatgttcaagtaccacctgaccgtggcccaagtccgcggaggcatggtgttcgagctggccaactccatcgtgctgcccttcgactgcagagactacgccgtggtgctgaggaagtacgccgacaaaatctactccatctccatgaagcacccccaggaaatgaagacctactccgtgtccttcgactccctgttctccgccgtgaagaatttcaccgagatcgcctccaagttcagcgagaggctgcaggacttcgacaagtccaacccaatcgtgctgaggatgatgaacgaccagctgatgttcctggaaagggccttcatcgaccccctgggcctgccagacagacccttctacaggcacgtgatctacgccccatcctcccacaacaaatacgccggcgagtccttccccggcatctacgatgccctgttcgacatcgagtccaaggtggacccctccaaggcctggggcgaagtgaagaggcaaatctacgtggccgccttcacagtgcaagccgctgccgaaaccctgtccgaggtggcctgaatcgcacctcgagatttaaatctgatcataatcagccataccacatttgtagaggttttacttgctttaaaaaacctcccacacctccccctgaacctgaaacataaaatgaatgcaattgttgttgttaacttgtttattgcagcttataatggttacaaataaagcaatagcatcacaaatttcacaaataaagcatttttttcactgcattctagttgtggtttgtccaaactcatcaatgtatcttatatgctggccaccgtacatgtggcttcccatgctcgcaagccctggcccgagttcgagcacaatgtcatgaccaggtgcaatatgcatctggggtcccgccgaggcatgttcatgccctaccagtgcaacctgaattatgtgaaggtgctgctggagcccgatgccatgtccagagtgagcctgacgggggtgtttgacatgaatgtggaggtgtggaagattctgagatatgatgaatccaagaccaggtgccgagcctgcgagtgcggagggaagcatgccaggttccagcccgtgtgtgtggatgtgacggaggacctgcgacccgatcatttggtgttgccctgcaccgggacggagttcggttccagcggggaagaatctgactagagtgagtagtgttctggggcgggggaggacctgcatgagggccagaataactgaaatctgtgcttttctgtgtgttgcagcagcatgagcggaagcggctcctttgagggaggggtattcagcccttatctgacggggcgtctcccctcctgggcgggagtgcgtcagaatgtgatgggatccacggtggacggccggcccgtgcagcccgcgaactcttcaaccctgacctatgcaaccctgagctcttcgtcgttggacgcagctgccgccgcagctgctgcatctgccgccagcgccgtgcgcggaatggccatgggcgccggctactacggcactctggtggccaactcgagttccaccaataatcccgccagcctgaacgaggagaagctgttgctgctgatggcccagctcgaggccttgacccagcgcctgggcgagctgacccagcaggtggctcagctgcaggagcagacgcgggccgcggttgccacggtgaaatccaaataaaaaatgaatcaataaataaacggagacggttgttgattttaacacagagtctgaatctttatttgatttttcgcgcgcggtaggccctggaccaccggtctcgatcattgagcacccggtggatcttttccaggacccggtagaggtgggcttggatgttgaggtacatgggcatgagcccgtcccgggggtggaggtagctccattgcagggcctcgtgctcgggggtggtgttgtaaatcacccagtcatagcaggggcgcagggcatggtgttgcacaatatctttgaggaggagactgatggccacgggcagccctttggtgtaggtgtttacaaatctgttgagctgggagggatgcatgcggggggagatgaggtgcatcttggcctggatcttgagattggcgatgttaccgcccagatcccgcctggggttcatgttgtgcaggaccaccagcacggtgtatccggtgcacttggggaatttatcatgcaacttggaagggaaggcgtgaaagaatttggcgacgcctttgtgcccgcccaggttttccatgcactcatccatgatgatggcgatgggcccgtgggcggcggcctgggcaaagacgtttcgggggtcggacacatcatagttgtggtcctgggtgaggtcatcataggccattttaatgaatttggggcggagggtgccggactgggggacaaaggtaccctcgatcccgggggcgtagttcccctcacagatctgcatctcccaggctttgagctcggagggggggatcatgtccacctgcggggcgataaagaacacggtttccggggcgggggagatgagctgggccgaaagcaagttccggagcagctgggacttgccgcagccggtggggccgtagatgaccccgatgaccggctgcaggtggtagttgagggagagacagctgccgtcctcccggaggaggggggccacctcgttcatcatctcgcgcacgtgcatgttctcgcgcaccagttccgccaggaggcgctctccccccagggataggagctcctggagcgaggcgaagtttttcagcggcttgagtccgtcggccatgggcattttggagagggtttgttgcaagagttccaggcggtcccagagctcggtgatgtgctctacggcatctcgatccagcagacctcctcgtttcgcgggttgggacggctgcgggagtagggcaccagacgatgggcgtccagcgcagccagggtccggtccttccagggtcgcagcgtccgcgtcagggtggtctccgtcacggtgaaggggtgcgcgccgggctgggcgcttgcgagggtgcgcttcaggctcatccggctggtcgaaaaccgctcccgatcggcgccctgcgcgtcggccaggtagcaattgaccatgagttcgtagttgagcgcctcggccgcgtggcctttggcgcggagcttacctttggaagtctgcccgcaggcgggacagaggagggacttgagggcgtagagcttgggggcgaggaagacggactcgggggcgtaggcgtccgcgccgcagtgggcgcagacggtctcgcactccacgagccaggtgaggtcgggctggtcggggtcaaaaaccagtttcccgccgttctttttgatgcgtttcttacctttggtctccatgagctcgtgtccccgctgggtgacaaagaggctgtccgtgtccccgtagaccgactttatgggccggtcctcgagcggtgtgccgcggtcctcctcgtagaggaaccccgcccactccgagacgaaagcccgggtccaggccagcacgaaggaggccacgtgggacgggtagcggtcgttgtccaccagcgggtccaccttttccagggtatgcaaacacatgtccccctcgtccacatccaggaaggtgattggcttgtaagtgtaggccacgtgaccgggggtcccggccgggggggtataaaagggtgcgggtccctgctcgtcctcactgtcttccggatcgctgtccaggagcgccagctgttggggtaggtattccctctcgaaggcgggcatgacctcggcactcaggttgtcagtttctagaaacgaggaggatttgatattgacggtgccggcggagatgcctttcaagagcccctcgtccatctggtcagaaaagacgatctttttgttgtcgagcttggtggcgaaggagccgtagagggcgttggagaggagcttggcgatggagcgcatggtctggtttttttccttgtcggcgcgctccttggcggcgatgttgagctgcacgtactcgcgcgccacgcacttccattcggggaagacggtggtcagctcgtcgggcacgattctgacctgccagccccgattatgcagggtgatgaggtccacactggtggccacctcgccgcgcaggggctcattagtccagcagaggcgtccgcccttgcgcgagcagaaggggggcagggggtccagcatgacctcgtcgggggggtcggcatcgatggtgaagatgccgggcaggaggtcggggtcaaagtagctgatggaagtggccagatcgtccagggcagcttgccattcgcgcacggccagcgcgcgctcgtagggactgaggggcgtgccccagggcatgggatgggtaagcgcggaggcgtacatgccgcagatgtcgtagacgtagaggggctcctcgaggatgccgatgtaggtggggtagcagcgccccccgcggatgctggcgcgcacgtagtcatacagctcgtgcgagggggcgaggagccccgggcccaggttggtgcgactgggcttttcggcgcggtagacgatctggcggaaaatggcatgcgagttggaggagatggtgggcctttggaagatgttgaagtgggcgtggggcagtccgaccgagtcgcggatgaagtgggcgtaggagtcttgcagcttggcgacgagctcggcggtgactaggacgtccagagcgcagtagtcgagggtctcctggatgatgtcatacttgagctgtcccttttgtttccacagctcgcggttgagaaggaactcttcgcggtccttccagtactcttcgagggggaacccgtcctgatctgcacggtaagagcctagcatgtagaactggttgacggccttgtaggcgcagcagcccttctccacggggagggcgtaggcctgggcggccttgcgcagggaggtgtgcgtgagggcgaaagtgtccctgaccatgaccttgaggaactggtgcttgaagtcgatatcgtcgcagcccccctgctcccagagctggaagtccgtgcgcttcttgtaggcggggttgggcaaagcgaaagtaacatcgttgaagaggatcttgcccgcgcggggcataaagttgcgagtgatgcggaaaggttggggcacctcggcccggttgttgatgacctgggcggcgagcacgatctcgtcgaagccgttgatgttgtggcccacgatgtagagttccacgaatcgcggacggcccttgacgtggggcagtttcttgagctcctcgtaggtgagctcgtcggggtcgctgagcccgtgctgctcgagcgcccagtcggcgagatgggggttggcgcggaggaaggaagtccagagatccacggccagggcggtttgcagacggtcccggtactgacggaactgctgcccgacggccattttttcgggggtgacgcagtagaaggtgcgggggtccccgtgccagcgatcccatttgagctggagggcgagatcgagggcgagctcgacgagccggtcgtccccggagagtttcatgaccagcatgaaggggacgagctgcttgccgaaggaccccatccaggtgtaggtttccacatcgtaggtgaggaagagcctttcggtgcgaggatgcgagccgatggggaagaactggatctcctgccaccaattggaggaatggctgttgatgtgatggaagtagaaatgccgacggcgcgccgaacactcgtgcttgtgtttatacaagcggccacagtgctcgcaacgctgcacgggatgcacgtgctgcacgagctgtacctgagttcctttgacgaggaatttcagtgggaagtggagtcgtggcgcctgcatctcgtgctgtactacgtcgtggtggtcggcctggccctcttctgcctcgatggtggtcatgctgacgagcccgcgcgggaggcaggtccagacctcggcgcgagcgggtcggagagcgaggacgagggcgcgcaggccggagctgtccagggtcctgagacgctgcggagtcaggtcagtgggcagcggcggcgcgcggttgacttgcaggagtttttccagggcgcgcgggaggtccagatggtacttgatctccaccgcgccattggtggcgacgtcgatggcttgcagggtcccgtgcccctggggtgtgaccaccgtcccccgtttcttcttgggcggctggggcgacgggggcggtgcctcttccatggttagaagcggcggcgaggacgcgcgccgggcggcaggggcggctcggggcccggaggcaggggcggcaggggcacgtcggcgccgcgcgcgggtaggttctggtactgcgcccggagaagactggcgtgagcgacgacgcgacggttgacgtcctggatctgacgcctctgggtgaaggccacgggacccgtgagtttgaacctgaaagagagttcgacagaatcaatctcggtatcgttgacggcggcctgccgcaggatctcttgcacgtcgcccgagttgtcctggtaggcgatctcggtcatgaactgctcgatctcctcctcttgaaggtctccgcggccggcgcgctccacggtggccgcgaggtcgttggagatgcggcccatgagctgcgagaaggcgttcatgcccgcctcgttccagacgcggctgtagaccacgacgccctcgggatcgcgggcgcgcatgaccacctgggcgaggttgagctccacgtggcgcgtgaagaccgcgtagttgcagaggcgctggtagaggtagttgagcgtggtggcgatgtgctcggtgacgaagaaatacatgatccagcggcggagcggcatctcgctgacgtcgcccagcgcctccaaacgttccatggcctcgtaaaagtccacggcgaagttgaaaaactgggagttgcgcgccgagacggtcaactcctcctccagaagacggatgagctcggcgatggtggcgcgcacctcgcgctcgaaggcccccgggagttcctccacttcctcttcttcctcctccactaacatctcttctacttcctcctcaggcggcagtggtggcgggggagggggcctgcgtcgccggcggcgcacgggcagacggtcgatgaagcgctcgatggtctcgccgcgccggcgtcgcatggtctcggtgacggcgcgcccgtcctcgcggggccgcagcgtgaagacgccgccgcgcatctccaggtggccgggggggtccccgttgggcagggagagggcgctgacgatgcatcttatcaattgccccgtagggactccgcgcaaggacctgagcgtctcgagatccacgggatctgaaaaccgctgaacgaaggcttcgagccagtcgcagtcgcaaggtaggctgagcacggtttcttctggcgggtcatgttggttgggagcggggcgggcgatgctgctggtgatgaagttgaaataggcggttctgagacggcggatggtggcgaggagcaccaggtctttgggcccggcttgctggatgcgcagacggtcggccatgccccaggcgtggtcctgacacctggccaggtccttgtagtagtcctgcatgagccgctccacgggcacctcctcctcgcccgcgcggccgtgcatgcgcgtgagcccgaagccgcgctggggctggacgagcgccaggtcggcgacgacgcgctcggcgaggatggcttgctggatctgggtgagggtggtctggaagtcatcaaagtcgacgaagcggtggtaggctccggtgttgatggtgtaggagcagttggccatgacggaccagttgacggtctggtggcccggacgcacgagctcgtggtacttgaggcgcgagtaggcgcgcgtgtcgaagatgtagtcgttgcaggtgcgcaccaggtactggtagccgatgaggaagtgcggcggcggctggcggtagagcggccatcgctcggtggcgggggcgccgggcgcgaggtcctcgagcatggtgcggtggtagccgtagatgtacctggacatccaggtgatgccggcggcggtggtggaggcgcgcgggaactcgcggacgcggttccagatgttgcgcagcggcaggaagtagttcatggtgggcacggtctggcccgtgaggcgcgcgcagtcgtggatgctctatacgggcaaaaacgaaagcggtcagcggctcgactccgtggcctggaggctaagcgaacgggttgggctgcgcgtgtaccccggttcgaatctcgaatcaggctggagccgcagctaacgtggtattggcactcccgtctcgacccaagcctgcaccaaccctccaggatacggaggcgggtcgttttgcaacttttttttggaggccggatgagactagtaagcgcggaaagcggccgaccgcgatggctcgctgccgtagtctggagaagaatcgccagggttgcgttgcggtgtgccccggttcgaggccggccggattccgcggctaacgagggcgtggctgccccgtcgtttccaagaccccatagccagccgacttctccagttacggagcgagcccctcttttgttttgtttgtttttgccagatgcatcccgtactgcggcagatgcgcccccaccaccctccaccgcaacaacagccccctccacagccggcgcttctgcccccgccccagcagcaacttccagccacgaccgccgcggccgccgtgagcggggctggacagagttatgatcaccagctggccttggaagagggcgaggggctggcgcgcctgggggcgtcgtcgccggagcggcacccgcgcgtgcagatgaaaagggacgctcgcgaggcctacgtgcccaagcagaacctgttcagagacaggagcggcgaggagcccgaggagatgcgcgcggcccggttccacgcggggcgggagctgcggcgcggcctggaccgaaagagggtgctgagggacgaggatttcgaggcggacgagctgacggggatcagccccgcgcgcgcgcacgtggccgcggccaacctggtcacggcgtacgagcagaccgtgaaggaggagagcaacttccaaaaatccttcaacaaccacgtgcgcaccctgatcgcgcgcgaggaggtgaccctgggcctgatgcacctgtgggacctgctggaggccatcgtgcagaaccccaccagcaagccgctgacggcgcagctgttcctggtggtgcagcatagtcgggacaacgaagcgttcagggaggcgctgctgaatatcaccgagcccgagggccgctggctcctggacctggtgaacattctgcagagcatcgtggtgcaggagcgcgggctgccgctgtccgagaagctggcggccatcaacttctcggtgctgagtttgggcaagtactacgctaggaagatctacaagaccccgtacgtgcccatagacaaggaggtgaagatcgacgggttttacatgcgcatgaccctgaaagtgctgaccctgagcgacgatctgggggtgtaccgcaacgacaggatgcaccgtgcggtgagcgccagcaggcggcgcgagctgagcgaccaggagctgatgcatagtctgcagcgggccctgaccggggccgggaccgagggggagagctactttgacatgggcgcggacctgcactggcagcccagccgccgggccttggaggcggcggcaggaccctacgtagaagaggtggacgatgaggtggacgaggagggcgagtacctggaagactgatggcgcgaccgtatttttgctagatgcaacaacaacagccacctcctgatcccgcgatgcgggcggcgctgcagagccagccgtccggcattaactcctcggacgattggacccaggccatgcaacgcatcatggcgctgacgacccgcaaccccgaagcctttagacagcagccccaggccaaccggctctcggccatcctggaggccgtggtgccctcgcgctccaaccccacgcacgagaaggtcctggccatcgtgaacgcgctggtggagaacaaggccatccgcggcgacgaggccggcctggtgtacaacgcgctgctggagcgcgtggcccgctacaacagcaccaacgtgcagaccaacctggaccgcatggtgaccgacgtgcgcgaggccgtggcccagcgcgagcggttccaccgcgagtccaacctgggatccatggtggcgctgaacgccttcctcagcacccagcccgccaacgtgccccggggccaggaggactacaccaacttcatcagcgccctgcgcctgatggtgaccgaggtgccccagagcgaggtgtaccagtccgggccggactacttcttccagaccagtcgccagggcttgcagaccgtgaacctgagccaggctttcaagaacttgcagggcctgtggggcgtgcaggccccggtcggggaccgcgcgacggtgtcgagcctgctgacgccgaactcgcgcctgctgctgctgctggtggcccccttcacggacagcggcagcatcaaccgcaactcgtacctgggctacctgattaacctgtaccgcgaggccatcggccaggcgcacgtggacgagcagacctaccaggagatcacccacgtgagccgcgccctgggccaggacgacccgggcaacctggaagccaccctgaactttttgctgaccaaccggtcgcagaagatcccgccccagtacgcgctcagcaccgaggaggagcgcatcctgcgttacgtgcagcagagcgtgggcctgttcctgatgcaggagggggccacccccagcgccgcgctcgacatgaccgcgcgcaacatggagcccagcatgtacgccagcaaccgcccgttcatcaataaactgatggactacttgcatcgggcggccgccatgaactctgactatttcaccaacgccatcctgaatccccactggctcccgccgccggggttctacacgggcgagtacgacatgcccgaccccaatgacgggttcctgtgggacgatgtggacagcagcgtgttctccccccgaccgggtgctaacgagcgccccttgtggaagaaggaaggcagcgaccgacgcccgtcctcggcgctgtccggccgcgagggtgctgccgcggcggtgcccgaggccgccagtcctttcccgagcttgcccttctcgctgaacagtatccgcagcagcgagctgggcaggatcacgcgcccgcgcttgctgggcgaagaggagtacttgaatgactcgctgttgagacccgagcgggagaagaacttccccaataacgggatagaaagcctggtggacaagatgagccgctggaagacgtatgcgcaggagcacagggacgatccccgggcgtcgcagggggccacgagccggggcagcgccgcccgtaaacgccggtggcacgacaggcagcggggacagatgtgggacgatgaggactccgccgacgacagcagcgtgttggacttgggtgggagtggtaacccgttcgctcacctgcgcccccgtatcgggcgcatgatgtaagagaaaccgaaaataaatgatactcaccaaggccatggcgaccagcgtgcgttcgtttcttctctgttgttgttgtatctagtatgatgaggcgtgcgtacccggagggtcctcctccctcgtacgagagcgtgatgcagcaggcgatggcggcggcggcgatgcagcccccgctggaggctccttacgtgcccccgcggtacctggcgcctacggaggggcggaacagcattcgttactcggagctggcacccttgtacgataccacccggttgtacctggtggacaacaagtcggcggacatcgcctcgctgaactaccagaacgaccacagcaacttcctgaccaccgtggtgcagaacaatgacttcacccccacggaggccagcacccagaccatcaactttgacgagcgctcgcggtggggcggccagctgaaaaccatcatgcacaccaacatgcccaacgtgaacgagttcatgtacagcaacaagttcaaggcgcgggtgatggtctcccgcaagacccccaatggggtgacagtgacagaggattatgatggtagtcaggatgagctgaagtatgaatgggtggaatttgagctgcccgaaggcaacttctcggtgaccatgaccatcgacctgatgaacaacgccatcatcgacaattacttggcggtggggcggcagaacggggtgctggagagcgacatcggcgtgaagttcgacactaggaacttcaggctgggctgggaccccgtgaccgagctggtcatgcccggggtgtacaccaacgaggctttccatcccgatattgtcttgctgcccggctgcggggtggacttcaccgagagccgcctcagcaacctgctgggcattcgcaagaggcagcccttccaggaaggcttccagatcatgtacgaggatctggaggggggcaacatccccgcgctcctggatgtcgacgcctatgagaaaagcaaggaggatgcagcagctgaagcaactgcagccgtagctaccgcctctaccgaggtcaggggcgataattttgcaagcgccgcagcagtggcagcggccgaggcggctgaaaccgaaagtaagatagtcattcagccggtggagaaggatagcaagaacaggagctacaacgtactaccggacaagataaacaccgcctaccgcagctggtacctagcctacaactatggcgaccccgagaagggcgtgcgctcctggacgctgctcaccacctcggacgtcacctgcggcgtggagcaagtctactggtcgctgcccgacatgatgcaagacccggtcaccttccgctccacgcgtcaagttagcaactacccggtggtgggcgccgagctcctgcccgtctactccaagagcttcttcaacgagcaggccgtctactcgcagcagctgcgcgccttcacctcgcttacgcacgtcttcaaccgcttccccgagaaccagatcctcgtccgcccgcccgcgcccaccattaccaccgtcagtgaaaacgttcctgctctcacagatcacgggaccctgccgctgcgcagcagtatccggggagtccagcgcgtgaccgttactgacgccagacgccgcacctgcccctacgtctacaaggccctgggcatagtcgcgccgcgcgtcctctcgagccgcaccttctaaatgtccattctcatctcgcccagtaataacaccggttggggcctgcgcgcgcccagcaagatgtacggaggcgctcgccaacgctccacgcaacaccccgtgcgcgtgcgcgggcacttccgcgctccctggggcgccctcaagggccgcgtgcggtcgcgcaccaccgtcgacgacgtgatcgaccaggtggtggccgacgcgcgcaactacacccccgccgccgcgcccgtctccaccgtggacgccgtcatcgacagcgtggtggccgacgcgcgccggtacgcccgcgccaagagccggcggcggcgcatcgcccggcggcaccggagcacccccgccatgcgcgcggcgcgagccttgctgcgcagggccaggcgcacgggacgcagggccatgctcagggcggccagacgcgcggcttcaggcgccagcgccggcaggacccggagacgcgcggccacggcggcggcagcggccatcgccagcatgtcccgcccgcggcgagggaacgtgtactgggtgcgcgacgccgccaccggtgtgcgcgtgcccgtgcgcacccgcccccctcgcacttgaagatgttcacttcgcgatgttgatgtgtcccagcggcgaggaggatgtccaagcgcaaattcaaggaagagatgctccaggtcatcgcgcctgagatctacggccctgcggtggtgaaggaggaaagaaagccccgcaaaatcaagcgggtcaaaaaggacaaaaaggaagaagaaagtgatgtggacggattggtggagtttgtgcgcgagttcgccccccggcggcgcgtgcagtggcgcgggcggaaggtgcaaccggtgctgagacccggcaccaccgtggtcttcacgcccggcgagcgctccggcaccgcttccaagcgctcctacgacgaggtgtacggggatgatgatattctggagcaggcggccgagcgcctgggcgagtttgcttacggcaagcgcagccgttccgcaccgaaggaagaggcggtgtccatcccgctggaccacggcaaccccacgccgagcctcaagcccgtgaccttgcagcaggtgctgccgaccgcggcgccgcgccgggggttcaagcgcgagggcgaggatctgtaccccaccatgcagctgatggtgcccaagcgccagaagctggaagacgtgctggagaccatgaaggtggacccggacgtgcagcccgaggtcaaggtgcggcccatcaagcaggtggccccgggcctgggcgtgcagaccgtggacatcaagattcccacggagcccatggaaacgcagaccgagcccatgatcaagcccagcaccagcaccatggaggtgcagacggatccctggatgccatcggctcctagtcgaagaccccggcgcaagtacggcgcggccagcctgctgatgcccaactacgcgctgcatccttccatcatccccacgccgggctaccgcggcacgcgcttctaccgcggtcataccagcagccgccgccgcaagaccaccactcgccgccgccgtcgccgcaccgccgctgcaaccacccctgccgccctggtgcggagagtgtaccgccgcggccgcgcacctctgaccctgccgcgcgcgcgctaccacccgagcatcgccatttaaactttcgcctgctttgcagatcaatggccctcacatgccgccttcgcgttcccattacgggctaccgaggaagaaaaccgcgccgtagaaggctggcggggaacgggatgcgtcgccaccaccaccggcggcggcgcgccatcagcaagcggttggggggaggcttcctgcccgcgctgatccccatcatcgccgcggcgatcggggcgatccccggcattgcttccgtggcggtgcaggcctctcagcgccactgagacacacttggaaacatcttgtaataaaccaatggactctgacgctcctggtcctgtgatgtgttttcgtagacagatggaagacatcaatttttcgtccctggctccgcgacacggcacgcggccgttcatgggcacctggagcgacatcggcaccagccaactgaacgggggcgccttcaattggagcagtctctggagcgggcttaagaatttcgggtccacgcttaaaacctatggcagcaaggcgtggaacagcaccacagggcaggcgctgagggataagctgaaagagcagaacttccagcagaaggtggtcgatgggctcgcctcgggcatcaacggggtggtggacctggccaaccaggccgtgcagcggcagatcaacagccgcctggacccggtgccgcccgccggctccgtggagatgccgcaggtggaggaggagctgcctcccctggacaagcggggcgagaagcgaccccgccccgatgcggaggagacgctgctgacgcacacggacgagccgcccccgtacgaggaggcggtgaaactgggtctgcccaccacgcggcccatcgcgcccctggccaccggggtgctgaaacccgaaaagcccgcgaccctggacttgcctcctccccagccttcccgcccctctacagtggctaagcccctgccgccggtggccgtggcccgcgcgcgacccgggggcaccgcccgccctcatgcgaactggcagagcactctgaacagcatcgtgggtctgggagtgcagagtgtgaagcgccgccgctgctattaaacctaccgtagcgcttaacttgcttgtctgtgtgtgtatgtattatgtcgccgccgccgctgtccaccagaaggaggagtgaagaggcgcgtcgccgagttgcaagatggccaccccatcgatgctgccccagtgggcgtacatgcacatcgccggacaggacgcttcggagtacctgagtccgggtctggtgcagtttgcccgcgccacagacacctacttcagtctggggaacaagtttaggaaccccacggtggcgcccacgcacgatgtgaccaccgaccgcagccagcggctgacgctgcgcttcgtgcccgtggaccgcgaggacaacacctactcgtacaaagtgcgctacacgctggccgtgggcgacaaccgcgtgctggacatggccagcacctactttgacatccgcggcgtgctggatcggggccctagcttcaaaccctactccggcaccgcctacaacagtctggcccccaagggagcacccaacacttgtcagtggacatataaagccgatggtgaaactgccacagaaaaaacctatacatatggaaatgcacccgtgcagggcattaacatcacaaaagatggtattcaacttggaactgacaccgatgatcagccaatctacgcagataaaacctatcagcctgaacctcaagtgggtgatgctgaatggcatgacatcactggtactgatgaaaagtatggaggcagagctcttaagcctgataccaaaatgaagccttgttatggttcttttgccaagcctactaataaagaaggaggtcaggcaaatgtgaaaacaggaacaggcactactaaagaatatgacatagacatggctttctttgacaacagaagtgcggctgctgctggcctagctccagaaattgttttgtatactgaaaatgtggatttggaaactccagatacccatattgtatacaaagcaggcacagatgacagcagctcttctattaatttgggtcagcaagccatgcccaacagacctaactacattggtttcagagacaactttatcgggctcatgtactacaacagcactggcaatatgggggtgctggccggtcaggcttctcagctgaatgctgtggttgacttgcaagacagaaacaccgagctgtcctaccagctcttgcttgactctctgggtgacagaacccggtatttcagtatgtggaatcaggcggtggacagctatgatcctgatgtgcgcattattgaaaatcatggtgtggaggatgaacttcccaactattgtttccctctggatgctgttggcagaacagatacttatcagggaattaaggctaatggaactgatcaaaccacatggaccaaagatgacagtgtcaatgatgctaatgagataggcaagggtaatccattcgccatggaaatcaacatccaagccaacctgtggaggaacttcctctacgccaacgtggccctgtacctgcccgactcttacaagtacacgccggccaatgttaccctgcccaccaacaccaacacctacgattacatgaacggccgggtggtggcgccctcgctggtggactcctacatcaacatcggggcgcgctggtcgctggatcccatggacaacgtgaaccccttcaaccaccaccgcaatgcggggctgcgctaccgctccatgctcctgggcaacgggcgctacgtgcccttccacatccaggtgccccagaaatttttcgccatcaagagcctcctgctcctgcccgggtcctacacctacgagtggaacttccgcaaggacgtcaacatgatcctgcagagctccctcggcaacgacctgcgcacggacggggcctccatctccttcaccagcatcaacctctacgccaccttcttccccatggcgcacaacacggcctccacgctcgaggccatgctgcgcaacgacaccaacgaccagtccttcaacgactacctctcggcggccaacatgctctaccccatcccggccaacgccaccaacgtgcccatctccatcccctcgcgcaactgggccgccttccgcggctggtccttcacgcgtctcaagaccaaggagacgccctcgctgggctccgggttcgacccctacttcgtctactcgggctccatcccctacctcgacggcaccttctacctcaaccacaccttcaagaaggtctccatcaccttcgactcctccgtcagctggcccggcaacgaccggctcctgacgcccaacgagttcgaaatcaagcgcaccgtcgacggcgagggctacaacgtggcccagtgcaacatgaccaaggactggttcctggtccagatgctggcccactacaacatcggctaccagggcttctacgtgcccgagggctacaaggaccgcatgtactccttcttccgcaacttccagcccatgagccgccaggtggtggacgaggtcaactacaaggactaccaggccgtcaccctggcctaccagcacaacaactcgggcttcgtcggctacctcgcgcccaccatgcgccagggccagccctaccccgccaactacccctacccgctcatcggcaagagcgccgtcaccagcgtcacccagaaaaagttcctctgcgacagggtcatgtggcgcatccccttctccagcaacttcatgtccatgggcgcgctcaccgacctcggccagaacatgctctatgccaactccgcccacgcgctagacatgaatttcgaagtcgaccccatggatgagtccacccttctctatgttgtcttcgaagtcttcgacgtcgtccgagtgcaccagccccaccgcggcgtcatcgaggccgtctacctgcgcacccccttctcggccggtaacgccaccacctaagctcttgcttcttgcaagccatggccgcgggctccggcgagcaggagctcagggccatcatccgcgacctgggctgcgggccctacttcctgggcaccttcgataagcgcttcccgggattcatggccccgcacaagctggcctgcgccatcgtcaacacggccggccgcgagaccgggggcgagcactggctggccttcgcctggaacccgcgctcgaacacctgctacctcttcgaccccttcgggttctcggacgagcgcctcaagcagatctaccagttcgagtacgagggcctgctgcgccgcagcgccctggccaccgaggaccgctgcgtcaccctggaaaagtccacccagaccgtgcagggtccgcgctcggccgcctgcgggctcttctgctgcatgttcctgcacgccttcgtgcactggcccgaccgccccatggacaagaaccccaccatgaacttgctgacgggggtgcccaacggcatgctccagtcgccccaggtggaacccaccctgcgccgcaaccaggaggcgctctaccgcttcctcaactcccactccgcctactttcgctcccaccgcgcgcgcatcgagaaggccaccgccttcgaccgcatgaatcaagacatgtaaaccgtgtgtgtatgttaaatgtctttaataaacagcactttcatgttacacatgcatctgagatgatttatttagaaatcgaaagggttctgccgggtctcggcatggcccgcgggcagggacacgttgcggaactggtacttggccagccacttgaactcggggatcagcagtttgggcagcggggtgtcggggaaggagtcggtccacagcttccgcgtcagttgcagggcgcccagcaggtcgggcgcggagatcttgaaatcgcagttgggacccgcgttctgcgcgcgggagttgcggtacacggggttgcagcactggaacaccatcagggccgggtgcttcacgctcgccagcaccgtcgcgtcggtgatgctctccacgtcgaggtcctcggcgttggccatcccgaagggggtcatcttgcaggtctgccttcccatggtgggcacgcacccgggcttgtggttgcaatcgcagtgcagggggatcagcatcatctgggcctggtcggcgttcatccccgggtacatggccttcatgaaagcctccaattgcctgaacgcctgctgggccttggctccctcggtgaagaagaccccgcaggacttgctagagaactggttggtggcgcacccggcgtcgtgcacgcagcagcgcgcgtcgttgttggccagctgcaccacgctgcgcccccagcggttctgggtgatcttggcccggtcggggttctccttcagcgcgcgctgcccgttctcgctcgccacatccatctcgatcatgtgctccttctggatcatggtggtcccgtgcaggcaccgcagcttgccctcggcctcggtgcacccgtgcagccacagcgcgcacccggtgcactcccagttcttgtgggcgatctgggaatgcgcgtgcacgaagccctgcaggaagcggcccatcatggtggtcagggtcttgttgctagtgaaggtcagcggaatgccgcggtgctcctcgttgatgtacaggtggcagatgcggcggtacacctcgccctgctcgggcatcagctggaagttggctttcaggtcggtctccacgcggtagcggtccatcagcatagtcatgatttccatacccttctcccaggccgagacgatgggcaggctcatagggttcttcaccatcatcttagcgctagcagccgcggccagggggtcgctctcgtccagggtctcaaagctccgcttgccgtccttctcggtgatccgcaccggggggtagctgaagcccacggccgccagctcctcctcggcctgtctttcgtcctcgctgtcctggctgacgtcctgcaggaccacatgcttggtcttgcggggtttcttcttgggcggcagcggcggcggagatgttggagatggcgagggggagcgcgagttctcgctcaccactactatctcttcctcttcttggtccgaggccacgcggcggtaggtatgtctcttcgggggcagaggcggaggcgacgggctctcgccgccgcgacttggcggatggctggcagagccccttccgcgttcgggggtgcgctcccggcggcgctctgactgacttcctccgcggccggccattgtgttctcctagggaggaacaacaagcatggagactcagccatcgccaacctcgccatctgcccccaccgccgacgagaagcagcagcagcagaatgaaagcttaaccgccccgccgcccagccccgccacctccgacgcggccgtcccagacatgcaagagatggaggaatccatcgagattgacctgggctatgtgacgcccgcggagcacgaggaggagctggcagtgcgcttttcacaagaagagatacaccaagaacagccagagcaggaagcagagaatgagcagagtcaggctgggctcgagcatgacggcgactacctccacctgagcgggggggaggacgcgctcatcaagcatctggcccggcaggccaccatcgtcaaggatgcgctgctcgaccgcaccgaggtgcccctcagcgtggaggagctcagccgcgcctacgagttgaacctcttctcgccgcgcgtgccccccaagcgccagcccaatggcacctgcgagcccaacccgcgcctcaacttctacccggtcttcgcggtgcccgaggccctggccacctaccacatctttttcaagaaccaaaagatccccgtctcctgccgcgccaaccgcacccgcgccgacgcccttttcaacctgggtcccggcgcccgcctacctgatatcgcctccttggaagaggttcccaagatcttcgagggtctgggcagcgacgagactcgggccgcgaacgctctgcaaggagaaggaggagagcatgagcaccacagcgccctggtcgagttggaaggcgacaacgcgcggctggcggtgctcaaacgcacggtcgagctgacccatttcgcctacccggctctgaacctgccccccaaagtcatgagcgcggtcatggaccaggtgctcatcaagcgcgcgtcgcccatctccgaggacgagggcatgcaagactccgaggagggcaagcccgtggtcagcgacgagcagctggcccggtggctgggtcctaatgctagtccccagagtttggaagagcggcgcaaactcatgatggccgtggtcctggtgaccgtggagctggagtgcctgcgccgcttcttcgccgacgcggagaccctgcgcaaggtcgaggagaacctgcactacctcttcaggcacgggttcgtgcgccaggcctgcaagatctccaacgtggagctgaccaacctggtctcctacatgggcatcttgcacgagaaccgcctggggcagaacgtgctgcacaccaccctgcgcggggaggcccggcgcgactacatccgcgactgcgtctacctctacctctgccacacctggcagacgggcatgggcgtgtggcagcagtgtctggaggagcagaacctgaaagagctctgcaagctcctgcagaagaacctcaagggtctgtggaccgggttcgacgagcgcaccaccgcctcggacctggccgacctcattttccccgagcgcctcaggctgacgctgcgcaacggcctgcccgactttatgagccaaagcatgttgcaaaactttcgctctttcatcctcgaacgctccggaatcctgcccgccacctgctccgcgctgccctcggacttcgtgccgctgaccttccgcgagtgccccccgccgctgtggagccactgctacctgctgcgcctggccaactacctggcctaccactcggacgtgatcgaggacgtcagcggcgagggcctgctcgagtgccactgccgctgcaacctctgcacgccgcaccgctccctggcctgcaacccccagctgctgagcgagacccagatcatcggcaccttcgagttgcaagggcccagcgaaggcgagggttcagccgccaaggggggtctgaaactcaccccggggctgtggacctcggcctacttgcgcaagttcgtgcccgaggactaccatcccttcgagatcaggttctacgaggaccaatcccatccgcccaaggccgagctgtcggcctgcgtcatcacccagggggcgatcctggcccaattgcaagccatccagaaatcccgccaagaattcttgctgaaaaagggccgcggggtctacctcgacccccagaccggtgaggagctcaaccccggcttcccccaggatgccccgaggaaacaagaagctgaaagtggagctgccgcccgtggaggatttggaggaagactgggagaacagcagtcaggcagaggaggaggagatggaggaagactgggacagcactcaggcagaggaggacagcctgcaagacagtctggaggaagacgaggaggaggcagaggaggaggtggaagaagcagccgccgccagaccgtcgtcctcggcgggggagaaagcaagcagcacggataccatctccgctccgggtcggggtcccgctcgaccacacagtagatgggacgagaccggacgattcccgaaccccaccacccagaccggtaagaaggagcggcagggatacaagtcctggcgggggcacaaaaacgccatcgtctcctgcttgcaggcctgcgggggcaacatctccttcacccggcgctacctgctcttccaccgcggggtgaactttccccgcaacatcttgcattactaccgtcacctccacagcccctactacttccaagaagaggcagcagcagcagaaaaagaccagcagaaaaccagcagctagaaaatccacagcggcggcagcaggtggactgaggatcgcggcgaacgagccggcgcaaacccgggagctgaggaaccggatctttcccaccctctatgccatcttccagcagagtcgggggcaggagcaggaactgaaagtcaagaaccgttctctgcgctcgctcacccgcagttgtctgtatcacaagagcgaagaccaacttcagcgcactctcgaggacgccgaggctctcttcaacaagtactgcgcgctcactcttaaagagtagcccgcgcccgcccagtcgcagaaaaaggcgggaattacgtcacctgtgcccttcgccctagccgcctccacccatcatcatgagcaaagagattcccacgccttacatgtggagctaccagccccagatgggcctggccgccggtgccgcccaggactactccacccgcatgaattggctcagcgccgggcccgcgatgatctcacgggtgaatgacatccgcgcccaccgaaaccagatactcctagaacagtcagcgctcaccgccacgccccgcaatcacctcaatccgcgtaattggcccgccgccctggtgtaccaggaaattccccagcccacgaccgtactacttccgcgagacgcccaggccgaagtccagctgactaactcaggtgtccagctggcgggcggcgccaccctgtgtcgtcaccgccccgctcagggtataaagcggctggtgatccggggcagaggcacacagctcaacgacgaggtggtgagctcttcgctgggtctgcgacctgacggagtcttccaactcgccggatcggggagatcttccttcacgcctcgtcaggccgtcctgactttggagagttcgtcctcgcagccccgctcgggtggcatcggcactctccagttcgtggaggagttcactccctcggtctacttcaaccccttctccggctcccccggccactacccggacgagttcatcccgaacttcgacgccatcagcgagtcggtggacggctacgattgaatgtcccatggtggcgcagctgacctagctcggcttcgacacctggaccactgccgccgcttccgctgcttcgctcgggatctcgccgagtttgcctactttgagctgcccgaggagcaccctcagggcccggcccacggagtgcggatcgtcgtcgaagggggcctcgactcccacctgcttcggatcttcagccagcgtccgatcctggtcgagcgcgagcaaggacagacccttctgactctgtactgcatctgcaaccaccccggcctgcatgaaagtctttgttgtctgctgtgtactgagtataataaaagctgagatcagcgactactccggacttccgtgtgttcctgaatccatcaaccagtctttgttcttcaccgggaacgagaccgagctccagctccagtgtaagccccacaagaagtacctcacctggctgttccagggctccccgatcgccgttgtcaaccactgcgacaacgacggagtcctgctgagcggccctgccaaccttactttttccacccgcagaagcaagctccagctcttccaacccttcctccccgggacctatcagtgcgtctcgggaccctgccatcacaccttccacctgatcccgaataccacagcgtcgctccccgctactaacaaccaaactaacctccaccaacgccaccgtcgctaggccacaatacatgcccatattagactatgaggccgagccacagcgacccatgctccccgctattagttacttcaatctaaccggcggagatgactgacccactggccaacaacaacgtcaacgaccttctcctggacatggacggccgcgcctcggagcagcgactcgcccaacttcgcattcgccagcagcaggagagagccgtcaaggagctgcaggatgcggtggccatccaccagtgcaagagaggcatcttctgcctggtgaaacaggccaagatctcctacgaggtcactccaaacgaccatcgcctctcctacgagctcctgcagcagcgccagaagttcacctgcctggtcggagtcaaccccatcgtcatcacccagcagtctggcgataccaaggggtgcatccactgctcctgcgactcccccgactgcgtccacactctgatcaagaccctctgcggcctccgcgacctcctccccatgaactaatcacccccttatccagtgaaataaagatcatattgatgatgattttacagaaataaaaaataatcatttgatttgaaataaagatacaatcatattgatgatttgagtttaacaaaaaaataaagaatcacttacttgaaatctgataccaggtctctgtccatgttttctgccaacaccacttcactcccctcttcccagctctggtactgcaggccccggcgggctgcaaacttcctccacacgctgaaggggatgtcaaattcctcctgtccctcaatcttcattttatcttctatcagatgtccaaaaagcgcgtccgggtggatgatgacttcgaccccgtctacccctacgatgcagacaacgcaccgaccgtgcccttcatcaacccccccttcgtctcttcagatggattccaagagaagcccctgggggtgttgtccctgcgactggccgaccccgtcaccaccaagaacggggaaatcaccctcaagctgggagagggggtggacctcgattcctcgggaaaactcatctccaacacggccaccaaggccgccgcccctctcagtttttccaacaacaccatttcccttaacatggatcaccccttttacactaaagatggaaaattatccttacaagtttctccaccattaaatatactgagaacaagcattctaaacacactagctttaggttttggatcaggtttaggactccgtggctctgccttggcagtacagttagtctctccacttacatttgatactgatggaaacataaagcttaccttagacagaggtttgcatgttacaacaggagatgcaattgaaagcaacataagctgggctaaaggtttaaaatttgaagatggagccatagcaaccaacattggaaatgggttagagtttggaagcagtagtacagaaacaggtgttgatgatgcttacccaatccaagttaaacttggatctggccttagctttgacagtacaggagccataatggctggtaacaaagaagacgataaactcactttgtggacaacacctgatccatcaccaaactgtcaaatactcgcagaaaatgatgcaaaactaacactttgcttgactaaatgtggtagtcaaatactggccactgtgtcagtcttagttgtaggaagtggaaacctaaaccccattactggcaccgtaagcagtgctcaggtgtttctacgttttgatgcaaacggtgttcttttaacagaacattctacactaaaaaaatactgggggtataggcagggagatagcatagatggcactccatataccaatgctgtaggattcatgcccaatttaaaagcttatccaaagtcacaaagttctactactaaaaataatatagtagggcaagtatacatgaatggagatgtttcaaaacctatgcttctcactataaccctcaatggtactgatgacagcaacagtacatattcaatgtcattttcatacacctggactaatggaagctatgttggagcaacatttggggctaactcttataccttctcatacatcgcccaagaatgaacactgtatcccaccctgcatgccaacccttcccaccccactctgtggaacaaactctgaaacacaaaataaaataaagttcaagtgttttattgattcaacagttttacaggattcgagcagttatttttcctccaccctcccaggacatggaatacaccaccctctccccccgcacagccttgaacatctgaatgccattggtgatggacatgcttttggtctccacgttccacacagtttcagagcgagccagtctcgggtcggtcagggagatgaaaccctccgggcactcccgcatctgcacctcacagctcaacagctgaggattgtcctcggtggtcgggatcacggttatctggaagaagcagaagagcggcggtgggaatcatagtccgcgaacgggatcggccggtggtgtcgcatcaggccccgcagcagtcgctgccgccgccgctccgtcaagctgctgctcagggggtccgggtccagggactccctcagcatgatgcccacggccctcagcatcagtcgtctggtgcggcgggcgcagcagcgcatgcggatctcgctcaggtcgctgcagtacgtgcaacacagaaccaccaggttgttcaacagtccatagttcaacacgctccagccgaaactcatcgcgggaaggatgctacccacgtggccgtcgtaccagatcctcaggtaaatcaagtggtgccccctccagaacacgctgcccacgtacatgatctccttgggcatgtggcggttcaccacctcccggtaccacatcaccctctggttgaacatgcagccccggatgatcctgcggaaccacagggccagcaccgccccgcccgccatgcagcgaagagaccccgggtcccggcaatggcaatggaggacccaccgctcgtacccgtggatcatctgggagctgaacaagtctatgttggcacagcacaggcatatgctcatgcatctcttcagcactctcaactcctcgggggtcaaaaccatatcccagggcacggggaactcttgcaggacagcgaaccccgcagaacagggcaatcctcgcacagaacttacattgtgcatggacagggtatcgcaatcaggcagcaccgggtgatcctccaccagagaagcgcgggtctcggtctcctcacagcgtggtaagggggccggccgatacgggtgatggcgggacgcggctgatcgtgttcgcgaccgtgtcatgatgcagttgctttcggacattttcgtacttgctgtagcagaacctggtccgggcgctgcacaccgatcgccggcggcggtctcggcgcttggaacgctcggtgttgaaattgtaaaacagccactctctcagaccgtgcagcagatctagggcctcaggagtgatgaagatcccatcatgcctgatggctctgatcacatcgaccaccgtggaatgggccagacccagccagatgatgcaattttgttgggtttcggtgacggcgggggagggaagaacaggaagaaccatgattaacttttaatccaaacggtctcggagtacttcaaaatgaagatcgcggagatggcacctctcgcccccgctgtgttggtggaaaataacagccaggtcaaaggtgatacggttctcgagatgttccacggtggcttccagcaaagcctccacgcgcacatccagaaacaagacaatagcgaaagcgggagggttctctaattcctcaatcatcatgttacactcctgcaccatccccagataattttcatttttccagccttgaatgattcgaactagttcctgaggtaaatccaagccagccatgataaagagctcgcgcagagcgccctccaccggcattcttaagcacaccctcataattccaagatattctgctcctggttcacctgcagcagattgacaagcggaatatcaaaatctctgccgcgatccctgagctcctccctcagcaataactgtaagtactctttcatatcctctccgaaatttttagccataggaccaccaggaataagattagggcaagccacagtacagataaaccgaagtcctccccagtgagcattgccaaatgcaagactgctataagcatgctggctagacccggtgatatcttccagataactggacagaaaatcgcccaggcaatttttaagaaaatcaacaaaagaaaaatcctccaggtggacgtttagagcctcgggaacaacgatgaagtaaatgcaagcggtgcgttccagcatggttagttagctgatctgtagaaaaaacaaaaatgaacattaaaccatgctagcctggcgaacaggtgggtaaatcgttctctccagcaccaggcaggccacggggtctccggcgcgaccctcgtaaaaattgtcgctatgattgaaaaccatcacagagagacgttcccggtggccggcgtgaatgattcgacaagatgaatacacccccggaacattggcgtccgcgagtgaaaaaaagcgcccgaggaagcaataaggcactacaatgctcagtctcaagtccagcaaagcgatgccatgcggatgaagcacaaaattctcaggtgcgtacaaaatgtaattactcccctcctgcacaggcagcaaagcccccgatccctccaggtacacatacaaagcctcagcgtccatagcttaccgagcagcagcacacaacaggcgcaagagtcagagaaaggctgagctctaacctgtccacccgctctctgctcaatatatagcccagatctacactgacgtaaaggccaaagtctaaaaatacccgccaaataatcacacacgcccagcacacgcccagaaaccggtgacacactcaaaaaaatacgcgcacttcctcaaacgcccaaaactgccgtcatttccgggttcccacgctacgtcatcaaaacacgactttcaaattccgtcgaccgttaaaaacgtcacccgccccgcccctaacggtcgcccgtctctcagccaatcagcgccccgcatccccaaattcaaacacctcatttgcatattaacgcgcacaaaaagtttgaggtatattattgatgatgg

SEQ ID NO: 45 - DNA, 34803 bp, synthetic construct
  misc_feature 1..34803: note = Synthetic Construct
  source 1..34803: mol_type = other DNA
ccatcttcaataatatacctcaaactttttgtgcgcgttaatatgcaaatgaggcgtttgaatttggggaggaagggcggtgattggtcgagggatgagcgaccgttaggggcggggcgagtgacgttttgatgacgtggttgcgaggaggagccagtttgcaagttctcgtgggaaaagtgacgtcaaacgaggtgtggtttgaacacggaaatactcaattttcccgcgctctctgacaggaaatgaggtgtttctgggcggatgcaagtgaaaacgggccattttcgcgcgaaaactgaatgaggaagtgaaaatctgagtaatttcgcgtttatggcagggaggagtatttgccgagggccgagtagactttgaccgattacgtgggggtttcgattaccgtgtttttcacctaaatttccgcgtacggtgtcaaagtccggtgtttttactactgtaatagtaatcaattacggggtcattagttcatagcccatatatggagttccgcgttacataacttacggtaaatggcccgcctggctgaccgcccaacgacccccgcccattgacgtcaataatgacgtatgttcccatagtaacgccaatagggactttccattgacgtcaatgggtggagtatttacggtaaactgcccacttggcagtacatcaagtgtatcatatgccaagtacgccccctattgacgtcaatgacggtaaatggcccgcctggcattatgcccagtacatgaccttatgggactttcctacttggcagtacatctacgtattagtcatcgctattaccatggtgatgcggttttggcagtacatcaatgggcgtggatagcggtttgactcacggggatttccaagtctccaccccattgacgtcaatgggagtttgttttggcaccaaaatcaacgggactttccaaaatgtcgtaacaactccgccccattgacgcaaatgggcggtaggcgtgtacggtgggaggtctatataagcagagctgtccctatcagtgatagagatctccctatcagtgatagagagtttagtgaaccgtcagatccgctagggtaccaacatggctagcatcgtcggagggtgggagtgcgaaaagcactcacagccatggcaggtcctggtcgcctcgcgcggacgcgccgtgtgtggaggtgtgctggtccacccgcagtgggtgttgactgcggcccattgcatcagaaataagtccgtgatcctcttggggagacattccctgtttcaccccgaagatactggacaggtgttccaagtgagccactccttcccgcatccactgtacgacatgagcctgctgaagaaccgctttctgcggccaggggacgactcatcacacgatttgatgctgcttcggctctcggaaccggccgagctcaccgacgcagtgaaggtcatggacctccctacgcaagagcctgctctcggtaccacttgttacgcatcgggatggggctccatcgagccggaagaattcctgaccccgaaaaagctgcagtgcgtggatctgcacgtgatttcgaatgacgtgtgcgcgcaagtgcatccacaaaaggtcactaagttcatgctgtgcgccggaaggtggaccggcggaaaatcgacctgttccggcgacagcggaggcccactcgtgtgcaacggtgtgctgcagggcatcactagctggggatcagaaccgtgcgcgcttccggagcggccctcgctctacacgaaggtggtgcactaccgcaaatggattaaagataccatcgtcgcaaaccctggatccgaaggtaggggttcattattgacctgtggagatgtcgaagaaaacccaggacccgctagcaaagcagtgctgctggcgctcctgatggctggactcgcgctgcagcctggaaccgccctgctctgttactcgtgcaaggcccaagtctcgaatgaggactgtttgcaagtggaaaactgcacccagctcggagaacaatgctggactgcacggatccgcgctgtcggcctgctgaccgtgatctccaaagggtgctcattgaactgcgtggacgatagccaggactactacgtgggaaagaagaatatcacttgttgcgacacggatctttgcaacgcgtccggagcgcacgccctgcagccagcagccgccattctggccctgcttccggccctggggttgctgctctggggtccgggccagctcggatcccagaccctgaactttgatctgctgaaactggcaggcgatgtggaaagcaacccaggcccaatggctagcgctcgcagaccgcggtggctgtgtgcaggggcgctcgtcctggcgggtggcttctttttgctcggctttcttttcggatggttcatcaaatcgtcaaacgaagctaccaatatcaccccgaagcacaacatgaaggcctttctggatgagctgaaggctgagaacattaagaagttcctctacaacttcacccagatcccacatttggcgggcactgagcagaactttcagttggctaagcagatccagagccagtggaaggaattcggcctggactccgtcgagctggcgcattacgatgtgctgctgagctaccctaataagactcatccgaactatatctcgattatcaatgaggacggaaacgaaatctttaacacgtccctcttcgagccgccaccgcctggatacgagaacgtgtcagatatcgtgcctccgttctcggccttctcgccccagggaatgcccgaaggggacctggtgtacgtgaactacgcaaggaccgaggacttcttcaagttggagcgggatatgaagatcaattgcagcggaaagatcgtcatcgcccgctacggcaaagtgttccgcggcaacaaggtgaagaatgcacagttggcaggcgccaagggcgtcatcctctactcggatcctgccgactacttcgctcctggcgtgaaatcctaccctgatggttggaatctgccaggaggaggggtgcagaggggaaatatcctgaacctgaacggtgccggtgacccacttactccgggttacccggccaacgaatacgcgtacaggcggggtatcgcggaagccgtcggactgccgtccatcccggtccatccgattggttactacgacgcccagaagctcctcgaaaagatgggaggcagcgcccctccggactcgtcatggagaggctcgctgaaggtgccatacaacgtgggacccggattcactggaaatttcagcactcaaaaagtgaagatgcacattcactccactaacgaagtcaccaggatctacaacgtcatcggaaccctccggggagcggtggaaccggaccgctacgtgatcctcggtggacaccgggatagctgggtgttcggaggaatcgatcctcaatcgggcgcagccgtcgtccatgaaatcgtcaggtcctttggtactcttaagaaggagggctggcgccctagacgcactattctgttcgcctcgtgggatgccgaagaatttggtctgctcggcagcaccgaatgggctgaggaaaactcccgcctgctccaagaacgcggagtggcgtacatcaatgccgactcatccatcgaaggaaactacacgctgcgggtggactgcactccactgatgtactcgctcgtgcacaacctgaccaaagaactcaaatccccagacgaaggattcgagggaaaatcgctgtacgagtcgtggaccaagaagagcccatccccggagttcagcgggatgccgcggatctcaaagctcggatcaggaaatgatttcgaagtgttctttcagaggctgggaattgcgtcgggaagggctcggtacacgaaaaactgggaaactaacaagttctcgggatacccgctgtaccactcggtgtatgaaacttacgaactggtggagaaattctacgatcctatgtttaagtaccacctgactgtggcccaagtgagaggcggaatggtgttcgagttggccaattcaattgtgctgccattcgattgccgcgactacgccgtggtgctgagaaagtacgcagacaaaatctactcaatcagcatgaagcacccacaagagatgaaaacctactcagtctccttcgactccctcttctccgcggtgaagaacttcaccgagatcgcgagcaaattctcggagcgccttcaagattttgacaaatccaatccgatcgtcctccgcatgatgaatgaccagctcatgtttctcgaacgggccttcatcgatccactgggacttccggaccggccgttttaccgccacgtgatctacgcgccctcgtcgcataacaagtatgctggagagagcttcccgggtatctacgacgcattgttcgacattgagtccaaggtggatccgtccaaagcctggggtgaagtgaagcgccaaatctacgtggcggcctttaccgtccaggcggcagcagaaaccttgagcgaggtggcttgactcgagcctaagcttctagataagatatccgatccaccggatctagataactgatcataatcagccataccacatttgtagaggttttacttgctttaaaaaacctcccacacctccccctgaacctgaaacataaaatgaatgcaattgttgttgttaacttgtttattgcagcttataatggttacaaataaagcaatagcatcacaaatttcacaaataaagcatttttttcactgcattctagttgtggtttgtccaaactcatcaatgtatcttatatgctggccaccgtacatgtggcttcccatgctcgcaagccctggcccgagttcgagcacaatgtcatgaccaggtgcaatatgcatctggggtcccgccgaggcatgttcatgccctaccagtgcaacctgaattatgtgaaggtgctgctggagcccgatgccatgtccagagtgagcctgacgggggtgtttgacatgaatgtggaggtgtggaagattctgagatatgatgaatccaagaccaggtgccgagcctgcgagtgcggagggaagcatgccaggttccagcccgtgtgtgtggatgtgacggaggacctgcgacccgatcatttggtgttgccctgcaccgggacggagttcggttccagcggggaagaatctgactagagtgagtagtgttctggggcgggggaggacctgcatgagggccagaataactgaaatctgtgcttttctgtgtgttgcagcagcatgagcggaagcggctcctttgagggaggggtattcagcccttatctgacggggcgtctcccctcctgggcgggagtgcgtcagaatgtgatgggatccacggtggacggccggcccgtgcagcccgcgaactcttcaaccctgacctatgcaaccctgagctcttcgtcgttggacgcagctgccgccgcagctgctgcatctgccgccagcgccgtgcgcggaatggccatgggcgccggctactacggcactctggtggccaactcgagttccaccaataatcccgccagcctgaacgaggagaagctgttgctgctgatggcccagctcgaggccttgacccagcgcctgggcgagctgacccagcaggtggctcagctgcaggagcagacgcgggccgcggttgccacggtgaaatccaaataaaaaatgaatcaataaataaacggagacggttgttgattttaacacagagtctgaatctttatttgatttttcgcgcgcggtaggccctggaccaccggtctcgatcattgagcacccggtggatcttttccaggacccggtagaggtgggcttggatgttgaggtacatgggcatgagcccgtcccgggggtggaggtagctccattgcagggcctcgtgctcgggggtggtgttgtaaatcacccagtcatagcaggggcgcagggcatggtgttgcacaatatctttgaggaggagactgatggccacgggcagccctttggtgtaggtgtttacaaatctgttgagctgggagggatgcatgcggggggagatgaggtgcatcttggcctggatcttgagattggcgatgttaccgcccagatcccgcctggggttcatgttgtgcaggaccaccagcacggtgtatccggtgcacttggggaatttatcatgcaacttggaagggaaggcgtgaaagaatttggcgacgcctttgtgcccgcccaggttttccatgcactcatccatgatgatggcgatgggcccgtgggcggcggcctgggcaaagacgtttcgggggtcggacacatcatagttgtggtcctgggtgaggtcatcataggccattttaatgaatttggggcggagggtgccggactgggggacaaaggtaccctcgatcccgggggcgtagttcccctcacagatctgcatctcccaggctttgagctcggagggggggatcatgtccacctgcggggcgataaagaacacggtttccggggcgggggagatgagctgggccgaaagcaagttccggagcagctgggacttgccgcagccggtggggccgtagatgaccccgatgaccggctgcaggtggtagttgagggagagacagctgccgtcctcccggaggaggggggccacctcgttcatcatctcgcgcacgtgcatgttctcgcgcaccagttccgccaggaggcgctctccccccagggataggagctcctggagcgaggcgaagtttttcagcggcttgagtccgtcggccatgggcattttggagagggtttgttgcaagagttccaggcggtcccagagctcggtgatgtgctctacggcatctcgatccagcagacctcctcgtttcgcgggttgggacggctgcgggagtagggcaccagacgatgggcgtccagcgcagccagggtccggtccttccagggtcgcagcgtccgcgtcagggtggtctccgtcacggtgaaggggtgcgcgccgggctgggcgcttgcgagggtgcgcttcaggctcatccggctggtcgaaaaccgctcccgatcggcgccctgcgcgtcggccaggtagcaattgaccatgagttcgtagttgagcgcctcggccgcgtggcctttggcgcggagcttacctttggaagtctgcccgcaggcgggacagaggagggacttgagggcgtagagcttgggggcgaggaagacggactcgggggcgtaggcgtccgcgccgcagtgggcgcagacggtctcgcactccacgagccaggtgaggtcgggctggtcggggtcaaaaaccagtttcccgccgttctttttgatgcgtttcttacctttggtctccatgagctcgtgtccccgctgggtgacaaagaggctgtccgtgtccccgtagaccgactttatgggccggtcctcgagcggtgtgccgcggtcctcctcgtagaggaaccccgcccactccgagacgaaagcccgggtccaggccagcacgaaggaggccacgtgggacgggtagcggtcgttgtccaccagcgggtccaccttttccagggtatgcaaacacatgtccccctcgtccacatccaggaaggtgattggcttgtaagtgtaggccacgtgaccgggggtcccggccgggggggtataaaagggtgcgggtccctgctcgtcctcactgtcttccggatcgctgtccaggagcgccagctgttggggtaggtattccctctcgaaggcgggcatgacctcggcactcaggttgtcagtttctagaaacgaggaggatttgatattgacggtgccggcggagatgcctttcaagagcccctcgtccatctggtcagaaaagacgatctttttgttgtcgagcttggtggcgaaggagccgtagagggcgttggagaggagcttggcgatggagcgcatggtctggtttttttccttgtcggcgcgctccttggcggcgatgttgagctgcacgtactcgcgcgccacgcacttccattcggggaagacggtggtcagctcgtcgggcacgattctgacctgccagccccgattatgcagggtgatgaggtccacactggtggccacctcgccgcgcaggggctcattagtccagcagaggcgtccgcccttgcgcgagcagaaggggggcagggggtccagcatgacctcgtcgggggggtcggcatcgatggtgaagatgccgggcaggaggtcggggtcaaagtagctgatggaagtggccagatcgtccagggcagcttgccattcgcgcacggccagcgcgcgctcgtagggactgaggggcgtgccccagggcatgggatgggtaagcgcggaggcgtacatgccgcagatgtcgtagacgtagaggggctcctcgaggatgccgatgtaggtggggtagcagcgccccccgcggatgctggcgcgcacgtagtcatacagctcgtgcgagggggcgaggagccccgggcccaggttggtgcgactgggcttttcggcgcggtagacgatctggcggaaaatggcatgcgagttggaggagatggtgggcctttggaagatgttgaagtgggcgtggggcagtccgaccgagtcgcggatgaagtgggcgtaggagtcttgcagcttggcgacgagctcggcggtgactaggacgtccagagcgcagtagtcgagggtctcctggatgatgtcatacttgagctgtcccttttgtttccacagctcgcggttgagaaggaactcttcgcggtccttccagtactcttcgagggggaacccgtcctgatctgcacggtaagagcctagcatgtagaactggttgacggccttgtaggcgcagcagcccttctccacggggagggcgtaggcctgggcggccttgcgcagggaggtgtgcgtgagggcgaaagtgtccctgaccatgaccttgaggaactggtgcttgaagtcgatatcgtcgcagcccccctgctcccagagctggaagtccgtgcgcttcttgtaggcggggttgggcaaagcgaaagtaacatcgttgaagaggatcttgcccgcgcggggcataaagttgcgagtgatgcggaaaggttggggcacctcggcccggttgttgatgacctgggcggcgagcacgatctcgtcgaagccgttgatgttgtggcccacgatgtagagttccacgaatcgcggacggcccttgacgtggggcagtttcttgagctcctcgtaggtgagctcgtcggggtcgctgagcccgtgctgctcgagcgcccagtcggcgagatgggggttggcgcggaggaaggaagtccagagatccacggccagggcggtttgcagacggtcccggtactgacggaactgctgcccgacggccattttttcgggggtgacgcagtagaaggtgcgggggtccccgtgccagcgatcccatttgagctggagggcgagatcgagggcgagctcgacgagccggtcgtccccggagagtttcatgaccagcatgaaggggacgagctgcttgccgaaggaccccatccaggtgtaggtttccacatcgtaggtgaggaagagcctttcggtgcgaggatgcgagccgatggggaagaactggatctcctgccaccaattggaggaatggctgttgatgtgatggaagtagaaatgccgacggcgcgccgaacactcgtgcttgtgtttatacaagcggccacagtgctcgcaacgctgcacgggatgcacgtgctgcacgagctgtacctgagttcctttgacgaggaatttcagtgggaagtggagtcgtggcgcctgcatctcgtgctgtactacgtcgtggtggtcggcctggccctcttctgcctcgatggtggtcatgctgacgagcccgcgcgggaggcaggtccagacctcggcgcgagcgggtcggagagcgaggacgagggcgcgcaggccggagctgtccagggtcctgagacgctgcggagtcaggtcagtgggcagcggcggcgcgcggttgacttgcaggagtttttccagggcgcgcgggaggtccagatggtacttgatctccaccgcgccattggtggcgacgtcgatggcttgcagggtcccgtgcccctggggtgtgaccaccgtcccccgtttcttcttgggcggctggggcgacgggggcggtgcctcttccatggttagaagcggcggcgaggacgcgcgccgggcggcaggggcggctcggggcccggaggcaggggcggcaggggcacgtcggcgccgcgcgcgggtaggttctggtactgcgcccggagaagactggcgtgagcgacgacgcgacggttgacgtcctggatctgacgcctctgggtgaaggccacgggacccgtgagtttgaacctgaaagagagttcgacagaatcaatctcggtatcgttgacggcggcctgccgcaggatctcttgcacgtcgcccgagttgtcctggtaggcgatctcggtcatgaactgctcgatctcctcctcttgaaggtctccgcggccggcgcgctccacggtggccgcgaggtcgttggagatgcggcccatgagctgcgagaaggcgttcatgcccgcctcgttccagacgcggctgtagaccacgacgccctcgggatcgcgggcgcgcatgaccacctgggcgaggttgagctccacgtggcgcgtgaagaccgcgtagttgcagaggcgctggtagaggtagttgagcgtggtggcgatgtgctcggtgacgaagaaatacatgatccagcggcggagcggcatctcgctgacgtcgcccagcgcctccaaacgttccatggcctcgtaaaagtccacggcgaagttgaaaaactgggagttgcgcgccgagacggtcaactcctcctccagaagacggatgagctcggcgatggtggcgcgcacctcgcgctcgaaggcccccgggagttcctccacttcctcttcttcctcctccactaacatctcttctacttcctcctcaggcggcagtggtggcgggggagggggcctgcgtcgccggcggcgcacgggcagacggtcgatgaagcgctcgatggtctcgccgcgccggcgtcgcatggtctcggtgacggcgcgcccgtcctcgcggggccgcagcgtgaagacgccgccgcgcatctccaggtggccgggggggtccccgttgggcagggagagggcgctgacgatgcatcttatcaattgccccgtagggactccgcgcaaggacctgagcgtctcgagatccacgggatctgaaaaccgctgaacgaaggcttcgagccagtcgcagtcgcaaggtaggctgagcacggtttcttctggcgggtcatgttggttgggagcggggcgggcgatgctgctggtgatgaagttgaaataggcggttctgagacggcggatggtggcgaggagcaccaggtctttgggcccggcttgctggatgcgcagacggtcggccatgccccaggcgtggtcctgacacctggccaggtccttgtagtagtcctgcatgagccgctccacgggcacctcctcctcgcccgcgcggccgtgcatgcgcgtgagcccgaagccgcgctggggctggacgagcgccaggtcggcgacgacgcgctcggcgaggatggcttgctggatctgggtgagggtggtctggaagtcatcaaagtcgacgaagcggtggtaggctccggtgttgatggtgtaggagcagttggccatgacggaccagttgacggtctggtggcccggacgcacgagctcgtggtacttgaggcgcgagtaggcgcgcgtgtcgaagatgtagtcgttgcaggtgcgcaccaggtactggtagccgatgaggaagtgcggcggcggctggcggtagagcggccatcgctcggtggcgggggcgccgggcgcgaggtcctcgagcatggtgcggtggtagccgtagatgtacctggacatccaggtgatgccggcggcggtggtggaggcgcgcgggaactcgcggacgcggttccagatgttgcgcagcggcaggaagtagttcatggtgggcacggtctggcccgtgaggcgcgcgcagtcgtggatgctctatacgggcaaaaacgaaagcggtcagcggctcgactccgtggcctggaggctaagcgaacgggttgggctgcgcgtgtaccccggttcgaatctcgaatcaggctggagccgcagctaacgtggtattggcactcccgtctcgacccaagcctgcaccaaccctccaggatacggaggcgggtcgttttgcaacttttttttggaggccggatgagactagtaagcgcggaaagcggccgaccgcgatggctcgctgccgtagtctggagaagaatcgccagggttgcgttgcggtgtgccccggttcgaggccggccggattccgcggctaacgagggcgtggctgccccgtcgtttccaagaccccatagccagccgacttctccagttacggagcgagcccctcttttgttttgtttgtttttgccagatgcatcccgtactgcggcagatgcgcccccaccaccctccaccgcaacaacagccccctccacagccggcgcttctgcccccgccccagcagcaacttccagccacgaccgccgcggccgccgtgagcggggctggacagagttatgatcaccagctggccttggaagagggcgaggggctggcgcgcctgggggcgtcgtcgccggagcggcacccgcgcgtgcagatgaaaagggacgctcgcgaggcctacgtgcccaagcagaacctgttcagagacaggagcggcgaggagcccgaggagatgcgcgcggcccggttccacgcggggcgggagctgcggcgcggcctggaccgaaagagggtgctgagggacgaggatttcgaggcggacgagctgacggggatcagccccgcgcgcgcgcacgtggccgcggccaacctggtcacggcgtacgagcagaccgtgaaggaggagagcaacttccaaaaatccttcaacaaccacgtgcgcaccctgatcgcgcgcgaggaggtgaccctgggcctgatgcacctgtgggacctgctggaggccatcgtgcagaaccccaccagcaagccgctgacggcgcagctgttcctggtggtgcagcatagtcgggacaacgaagcgttcagggaggcgctgctgaatatcaccgagcccgagggccgctggctcctggacctggtgaacattctgcagagcatcgtggtgcaggagcgcgggctgccgctgtccgagaagctggcggccatcaacttctcggtgctgagtttgggcaagtactacgctaggaagatctacaagaccccgtacgtgcccatagacaaggaggtgaagatcgacgggttttacatgcgcatgaccctgaaagtgctgaccctgagcgacgatctgggggtgtaccgcaacgacaggatgcaccgtgcggtgagcgccagcaggcggcgcgagctgagcgaccaggagctgatgcatagtctgcagcgggccctgaccggggccgggaccgagggggagagctactttgacatgggcgcggacctgcactggcagcccagccgccgggccttggaggcggcggcaggaccctacgtagaagaggtggacgatgaggtggacgaggagggcgagtacctggaagactgatggcgcgaccgtatttttgctagatgcaacaacaacagccacctcctgatcccgcgatgcgggcggcgctgcagagccagccgtccggcattaactcctcggacgattggacccaggccatgcaacgcatcatggcgctgacgacccgcaaccccgaagcctttagacagcagccccaggccaaccggctctcggccatcctggaggccgtggtgccctcgcgctccaaccccacgcacgagaaggtcctggccatcgtgaacgcgctggtggagaacaaggccatccgcggcgacgaggccggcctggtgtacaacgcgctgctggagcgcgtggcccgctacaacagcaccaacgtgcagaccaacctggaccgcatggtgaccgacgtgcgcgaggccgtggcccagcgcgagcggttccaccgcgagtccaacctgggatccatggtggcgctgaacgccttcctcagcacccagcccgccaacgtgccccggggccaggaggactacaccaacttcatcagcgccctgcgcctgatggtgaccgaggtgccccagagcgaggtgtaccagtccgggccggactacttcttccagaccagtcgccagggcttgcagaccgtgaacctgagccaggctttcaagaacttgcagggcctgtggggcgtgcaggccccggtcggggaccgcgcgacggtgtcgagcctgctgacgccgaactcgcgcctgctgctgctgctggtggcccccttcacggacagcggcagcatcaaccgcaactcgtacctgggctacctgattaacctgtaccgcgaggccatcggccaggcgcacgtggacgagcagacctaccaggagatcacccacgtgagccgcgccctgggccaggacgacccgggcaacctggaagccaccctgaactttttgctgaccaaccggtcgcagaagatcccgccccagtacgcgctcagcaccgaggaggagcgcatcctgcgttacgtgcagcagagcgtgggcctgttcctgatgcaggagggggccacccccagcgccgcgctcgacatgaccgcgcgcaacatggagcccagcatgtacgccagcaaccgcccgttcatcaataaactgatggactacttgcatcgggcggccgccatgaactctgactatttcaccaacgccatcctgaatccccactggctcccgccgccggggttctacacgggcgagtacgacatgcccgaccccaatgacgggttcctgtgggacgatgtggacagcagcgtgttctccccccgaccgggtgctaacgagcgccccttgtggaagaaggaaggcagcgaccgacgcccgtcctcggcgctgtccggccgcgagggtgctgccgcggcggtgcccgaggccgccagtcctttcccgagcttgcccttctcgctgaacagtatccgcagcagcgagctgggcaggatcacgcgcccgcgcttgctgggcgaagaggagtacttgaatgactcgctgttgagacccgagcgggagaagaacttccccaataacgggatagaaagcctggtggacaagatgagccgctggaagacgtatgcgcaggagcacagggacgatccccgggcgtcgcagggggccacgagccggggcagcgccgcccgtaaacgccggtggcacgacaggcagcggggacagatgtgggacgatgaggactccgccgacgacagcagcgtgttggacttgggtgggagtggtaacccgttcgctcacctgcgcccccgtatcgggcgcatgatgtaagagaaaccgaaaataaatgatactcaccaaggccatggcgaccagcgtgcgttcgtttcttctctgttgttgttgtatctagtatgatgaggcgtgcgtacccggagggtcctcctccctcgtacgagagcgtgatgcagcaggcgatggcggcggcggcgatgcagcccccgctggaggctccttacgtgcccccgcggtacctggcgcctacggaggggcggaacagcattcgttactcggagctggcacccttgtacgataccacccggttgtacctggtggacaacaagtcggcggacatcgcctcgctgaactaccagaacgaccacagcaacttcctgaccaccgtggtgcagaacaatgacttcacccccacggaggccagcacccagaccatcaactttgacgagcgctcgcggtggggcggccagctgaaaaccatcatgcacaccaacatgcccaacgtgaacgagttcatgtacagcaacaagttcaaggcgcgggtgatggtctcccgcaagacccccaatggggtgacagtgacagaggattatgatggtagtcaggatgagctgaagtatgaatgggtggaatttgagctgcccgaaggcaacttctcggtgaccatgaccatcgacctgatgaacaacgccatcatcgacaattacttggcggtggggcggcagaacggggtgctggagagcgacatcggcgtgaagttcgacactaggaacttcaggctgggctgggaccccgtgaccgagctggtcatgcccggggtgtacaccaacgaggctttccatcccgatattgtcttgctgcccggctgcggggtggacttcaccgagagccgcctcagcaacctgctgggcattcgcaagaggcagcccttccaggaaggcttccagatcatgtacgaggatctggaggggggcaacatccccgcgctcctggatgtcgacgcctatgagaaaagcaaggaggatgcagcagctgaagcaactgcagccgtagctaccgcctctaccgaggtcaggggcgataattttgcaagcgccgcagcagtggcagcggccgaggcggctgaaaccgaaagtaagatagtcattcagccggtggagaaggatagcaagaacaggagctacaacgtactaccggacaagataaacaccgcctaccgcagctggtacctagcctacaactatggcgaccccgagaagggcgtgcgctcctggacgctgctcaccacctcggacgtcacctgcggcgtggagcaagtctactggtcgctgcccgacatgatgcaagacccggtcaccttccgctccacgcgtcaagttagcaactacccggtggtgggcgccgagctcctgcccgtctactccaagagcttcttcaacgagcaggccgtctactcgcagcagctgcgcgccttcacctcgcttacgcacgtcttcaaccgcttccccgagaaccagatcctcgtccgcccgcccgcgcccaccattaccaccgtcagtgaaaacgttcctgctctcacagatcacgggaccctgccgctgcgcagcagtatccggggagtccagcgcgtgaccgttactgacgccagacgccgcacctgcccctacgtctacaaggccctgggcatagtcgcgccgcgcgtcctctcgagccgcaccttctaaatgtccattctcatctcgcccagtaataacaccggttggggcctgcgcgcgcccagcaagatgtacggaggcgctcgccaacgctccacgcaacaccccgtgcgcgtgcgcgggcacttccgcgctccctggggcgccctcaagggccgcgtgcggtcgcgcaccaccgtcgacgacgtgatcgaccaggtggtggccgacgcgcgcaactacacccccgccgccgcgcccgtctccaccgtggacgccgtcatcgacagcgtggtggccgacgcgcgccggtacgcccgcgccaagagccggcggcggcgcatcgcccggcggcaccggagcacccccgccatgcgcgcggcgcgagccttgctgcgcagggccaggcgcacgggacgcagggccatgctcagggcggccagacgcgcggcttcaggcgccagcgccggcaggacccggagacgcgcggccacggcggcggcagcggccatcgccagcatgtcccgcccgcggcgagggaacgtgtactgggtgcgcgacgccgccaccggtgtgcgcgtgcccgtgcgcacccgcccccctcgcacttgaagatgttcacttcgcgatgttgatgtgtcccagcggcgaggaggatgtccaagcgcaaattcaaggaagagatgctccaggtcatcgcgcctgagatctacggccctgcggtggtgaaggaggaaagaaagccccgcaaaatcaagcgggtcaaaaaggacaaaaaggaagaagaaagtgatgtggacggattggtggagtttgtgcgcgagttcgccccccggcggcgcgtgcagtggcgcgggcggaaggtgcaaccggtgctgagacccggcaccaccgtggtcttcacgcccggcgagcgctccggcaccgcttccaagcgctcctacgacgaggtgtacggggatgatgatattctggagcaggcggccgagcgcctgggcgagtttgcttacggcaagcgcagccgttccgcaccgaaggaagaggcggtgtccatcccgctggaccacggcaaccccacgccgagcctcaagcccgtgaccttgcagcaggtgctgccgaccgcggcgccgcgccgggggttcaagcgcgagggcgaggatctgtaccccaccatgcagctgatggtgcccaagcgccagaagctggaagacgtgctggagaccatgaaggtggacccggacgtgcagcccgaggtcaaggtgcggcccatcaagcaggtggccccgggcctgggcgtgcagaccgtggacatcaagattcccacggagcccatggaaacgcagaccgagcccatgatcaagcccagcaccagcaccatggaggtgcagacggatccctggatgccatcggctcctagtcgaagaccccggcgcaagtacggcgcggccagcctgctgatgcccaactacgcgctgcatccttccatcatccccacgccgggctaccgcggcacgcgcttctaccgcggtcataccagcagccgccgccgcaagaccaccactcgccgccgccgtcgccgcaccgccgctgcaaccacccctgccgccctggtgcggagagtgtaccgccgcggccgcgcacctctgaccctgccgcgcgcgcgctaccacccgagcatcgccatttaaactttcgcctgctttgcagatcaatggccctcacatgccgccttcgcgttcccattacgggctaccgaggaagaaaaccgcgccgtagaaggctggcggggaacgggatgcgtcgccaccaccaccggcggcggcgcgccatcagcaagcggttggggggaggcttcctgcccgcgctgatccccatcatcgccgcggcgatcggggcgatccccggcattgcttccgtggcggtgcaggcctctcagcgccactgagacacacttggaaacatcttgtaataaaccaatggactctgacgctcctggtcctgtgatgtgttttcgtagacagatggaagacatcaatttttcgtccctggctccgcgacacggcacgcggccgttcatgggcacctggagcgacatcggcaccagccaactgaacgggggcgccttcaattggagcagtctctggagcgggcttaagaatttcgggtccacgcttaaaacctatggcagcaaggcgtggaacagcaccacagggcaggcgctgagggataagctgaaagagcagaacttccagcagaaggtggtcgatgggctcgcctcgggcatcaacggggtggtggacctggccaaccaggccgtgcagcggcagatcaacagccgcctggacccggtgccgcccgccggctccgtggagatgccgcaggtggaggaggagctgcctcccctggacaagcggggcgagaagcgaccccgccccgatgcggaggagacgctgctgacgcacacggacgagccgcccccgtacgaggaggcggtgaaactgggtctgcccaccacgcggcccatcgcgcccctggccaccggggtgctgaaacccgaaaagcccgcgaccctggacttgcctcctccccagccttcccgcccctctacagtggctaagcccctgccgccggtggccgtggcccgcgcgcgacccgggggcaccgcccgccctcatgcgaactggcagagcactctgaacagcatcgtgggtctgggagtgcagagtgtgaagcgccgccgctgctattaaacctaccgtagcgcttaacttgcttgtctgtgtgtgtatgtattatgtcgccgccgccgctgtccaccagaaggaggagtgaagaggcgcgtcgccgagttgcaagatggccaccccatcgatgctgccccagtgggcgtacatgcacatcgccggacaggacgcttcggagtacctgagtccgggtctggtgcagtttgcccgcgccacagacacctacttcagtctggggaacaagtttaggaaccccacggtggcgcccacgcacgatgtgaccaccgaccgcagccagcggctgacgctgcgcttcgtgcccgtggaccgcgaggacaacacctactcgtacaaagtgcgctacacgctggccgtgggcgacaaccgcgtgctggacatggccagcacctactttgacatccgcggcgtgctggatcggggccctagcttcaaaccctactccggcaccgcctacaacagtctggcccccaagggagcacccaacacttgtcagtggacatataaagccgatggtgaaactgccacagaaaaaacctatacatatggaaatgcacccgtgcagggcattaacatcacaaaagatggtattcaacttggaactgacaccgatgatcagccaatctacgcagataaaacctatcagcctgaacctcaagtgggtgatgctgaatggcatgacatcactggtactgatgaaaagtatggaggcagagctcttaagcctgataccaaaatgaagccttgttatggttcttttgccaagcctactaataaagaaggaggtcaggcaaatgtgaaaacaggaacaggcactactaaagaatatgacatagacatggctttctttgacaacagaagtgcggctgctgctggcctagctccagaaattgttttgtatactgaaaatgtggatttggaaactccagatacccatattgtatacaaagcaggcacagatgacagcagctcttctattaatttgggtcagcaagccatgcccaacagacctaactacattggtttcagagacaactttatcgggctcatgtactacaacagcactggcaatatgggggtgctggccggtcaggcttctcagctgaatgctgtggttgacttgcaagacagaaacaccgagctgtcctaccagctcttgcttgactctctgggtgacagaacccggtatttcagtatgtggaatcaggcggtggacagctatgatcctgatgtgcgcattattgaaaatcatggtgtggaggatgaacttcccaactattgtttccctctggatgctgttggcagaacagatacttatcagggaattaaggctaatggaactgatcaaaccacatggaccaaagatgacagtgtcaatgatgctaatgagataggcaagggtaatccattcgccatggaaatcaacatccaagccaacctgtggaggaacttcctctacgccaacgtggccctgtacctgcccgactcttacaagtacacgccggccaatgttaccctgcccaccaacaccaacacctacgattacatgaacggccgggtggtggcgccctcgctggtggactcctacatcaacatcggggcgcgctggtcgctggatcccatggacaacgtgaaccccttcaaccaccaccgcaatgcggggctgcgctaccgctccatgctcctgggcaacgggcgctacgtgcccttccacatccaggtgccccagaaatttttcgccatcaagagcctcctgctcctgcccgggtcctacacctacgagtggaacttccgcaaggacgtcaacatgatcctgcagagctccctcggcaacgacctgcgcacggacggggcctccatctccttcaccagcatcaacctctacgccaccttcttccccatggcgcacaacacggcctccacgctcgaggccatgctgcgcaacgacaccaacgaccagtccttcaacgactacctctcggcggccaacatgctctaccccatcccggccaacgccaccaacgtgcccatctccatcccctcgcgcaactgggccgccttccgcggctggtccttcacgcgtctcaagaccaaggagacgccctcgctgggctccgggttcgacccctacttcgtctactcgggctccatcccctacctcgacggcaccttctacctcaaccacaccttcaagaaggtctccatcaccttcgactcctccgtcagctggcccggcaacgaccggctcctgacgcccaacgagttcgaaatcaagcgcaccgtcgacggcgagggctacaacgtggcccagtgcaacatgaccaaggactggttcctggtccagatgctggcccactacaacatcggctaccagggcttctacgtgcccgagggctacaaggaccgcatgtactccttcttccgcaacttccagcccatgagccgccaggtggtggacgaggtcaactacaaggactaccaggccgtcaccctggcctaccagcacaacaactcgggcttcgtcggctacctcgcgcccaccatgcgccagggccagccctaccccgccaactacccctacccgctcatcggcaagagcgccgtcaccagcgtcacccagaaaaagttcctctgcgacagggtcatgtggcgcatccccttctccagcaacttcatgtccatgggcgcgctcaccgacctcggccagaacatgctctatgccaactccgcccacgcgctagacatgaatttcgaagtcgaccccatggatgagtccacccttctctatgttgtcttcgaagtcttcgacgtcgtccgagtgcaccagccccaccgcggcgtcatcgaggccgtctacctgcgcacccccttctcggccggtaacgccaccacctaagctcttgcttcttgcaagccatggccgcgggctccggcgagcaggagctcagggccatcatccgcgacctgggctgcgggccctacttcctgggcaccttcgataagcgcttcccgggattcatggccccgcacaagctggcctgcgccatcgtcaacacggccggccgcgagaccgggggcgagcactggctggccttcgcctggaacccgcgctcgaacacctgctacctcttcgaccccttcgggttctcggacgagcgcctcaagcagatctaccagttcgagtacgagggcctgctgcgccgcagcgccctggccaccgaggaccgctgcgtcaccctggaaaagtccacccagaccgtgcagggtccgcgctcggccgcctgcgggctcttctgctgcatgttcctgcacgccttcgtgcactggcccgaccgccccatggacaagaaccccaccatgaacttgctgacgggggtgcccaacggcatgctccagtcgccccaggtggaacccaccctgcgccgcaaccaggaggcgctctaccgcttcctcaactcccactccgcctactttcgctcccaccgcgcgcgcatcgagaaggccaccgccttcgaccgcatgaatcaagacatgtaaaccgtgtgtgtatgttaaatgtctttaataaacagcactttcatgttacacatgcatctgagatgatttatttagaaatcgaaagggttctgccgggtctcggcatggcccgcgggcagggacacgttgcggaactggtacttggccagccacttgaactcggggatcagcagtttgggcagcggggtgtcggggaaggagtcggtccacagcttccgcgtcagttgcagggcgcccagcaggtcgggcgcggagatcttgaaatcgcagttgggacccgcgttctgcgcgcgggagttgcggtacacggggttgcagcactggaacaccatcagggccgggtgcttcacgctcgccagcaccgtcgcgtcggtgatgctctccacgtcgaggtcctcggcgttggccatcccgaagggggtcatcttgcaggtctgccttcccatggtgggcacgcacccgggcttgtggttgcaatcgcagtgcagggggatcagcatcatctgggcctggtcggcgttcatccccgggtacatggccttcatgaaagcctccaattgcctgaacgcctgctgggccttggctccctcggtgaagaagaccccgcaggacttgctagagaactggttggtggcgcacccggcgtcgtgcacgcagcagcgcgcgtcgttgttggccagctgcaccacgctgcgcccccagcggttctgggtgatcttggcccggtcggggttctccttcagcgcgcgctgcccgttctcgctcgccacatccatctcgatcatgtgctccttctggatcatggtggtcccgtgcaggcaccgcagcttgccctcggcctcggtgcacccgtgcagccacagcgcgcacccggtgcactcccagttcttgtgggcgatctgggaatgcgcgtgcacgaagccctgcaggaagcggcccatcatggtggtcagggtcttgttgctagtgaaggtcagcggaatgccgcggtgctcctcgttgatgtacaggtggcagatgcggcggtacacctcgccctgctcgggcatcagctggaagttggctttcaggtcggtctccacgcggtagcggtccatcagcatagtcatgatttccatacccttctcccaggccgagacgatgggcaggctcatagggttcttcaccatcatcttagcgctagcagccgcggccagggggtcgctctcgtccagggtctcaaagctccgcttgccgtccttctcggtgatccgcaccggggggtagctgaagcccacggccgccagctcctcctcggcctgtctttcgtcctcgctgtcctggctgacgtcctgcaggaccacatgcttggtcttgcggggtttcttcttgggcggcagcggcggcggagatgttggagatggcgagggggagcgcgagttctcgctcaccactactatctcttcctcttcttggtccgaggccacgcggcggtaggtatgtctcttcgggggcagaggcggaggcgacgggctctcgccgccgcgacttggcggatggctggcagagccccttccgcgttcgggggtgcgctcccggcggcgctctgactgacttcctccgcggccggccattgtgttctcctagggaggaacaacaagcatggagactcagccatcgccaacctcgccatctgcccccaccgccgacgagaagcagcagcagcagaatgaaagcttaaccgccccgccgcccagccccgccacctccgacgcggccgtcccagacatgcaagagatggaggaatccatcgagattgacctgggctatgtgacgcccgcggagcacgaggaggagctggcagtgcgcttttcacaagaagagatacaccaagaacagccagagcaggaagcagagaatgagcagagtcaggctgggctcgagcatgacggcgactacctccacctgagcgggggggaggacgcgctcatcaagcatctggcccggcaggccaccatcgtcaaggatgcgctgctcgaccgcaccgaggtgcccctcagcgtggaggagctcagccgcgcctacgagttgaacctcttctcgccgcgcgtgccccccaagcgccagcccaatggcacctgcgagcccaacccgcgcctcaacttctacccggtcttcgcggtgcccgaggccctggccacctaccacatctttttcaagaaccaaaagatccccgtctcctgccgcgccaaccgcacccgcgccgacgcccttttcaacctgggtcccggcgcccgcctacctgatatcgcctccttggaagaggttcccaagatcttcgagggtctgggcagcgacgagactcgggccgcgaacgctctgcaaggagaaggaggagagcatgagcaccacagcgccctggtcgagttggaaggcgacaacgcgcggctggcggtgctcaaacgcacggtcgagctgacccatttcgcctacccggctctgaacctgccccccaaagtcatgagcgcggtcatggaccaggtgctcatcaagcgcgcgtcgcccatctccgaggacgagggcatgcaagactccgaggagggcaagcccgtggtcagcgacgagcagctggcccggtggctgggtcctaatgctagtccccagagtttggaagagcggcgcaaactcatgatggccgtggtcctggtgaccgtggagctggagtgcctgcgccgcttcttcgccgacgcggagaccctgcgcaaggtcgaggagaacctgcactacctcttcaggcacgggttcgtgcgccaggcctgcaagatctccaacgtggagctgaccaacctggtctcctacatgggcatcttgcacgagaaccgcctggggcagaacgtgctgcacaccaccctgcgcggggaggcccggcgcgactacatccgcgactgcgtctacctctacctctgccacacctggcagacgggcatgggcgtgtggcagcagtgtctggaggagcagaacctgaaagagctctgcaagctcctgcagaagaacctcaagggtctgtggaccgggttcgacgagcgcaccaccgcctcggacctggccgacctcattttccccgagcgcctcaggctgacgctgcgcaacggcctgcccgactttatgagccaaagcatgttgcaaaactttcgctctttcatcctcgaacgctccggaatcctgcccgccacctgctccgcgctgccctcggacttcgtgccgctgaccttccgcgagtgccccccgccgctgtggagccactgctacctgctgcgcctggccaactacctggcctaccactcggacgtgatcgaggacgtcagcggcgagggcctgctcgagtgccactgccgctgcaacctctgcacgccgcaccgctccctggcctgcaacccccagctgctgagcgagacccagatcatcggcaccttcgagttgcaagggcccagcgaaggcgagggttcagccgccaaggggggtctgaaactcaccccggggctgtggacctcggcctacttgcgcaagttcgtgcccgaggactaccatcccttcgagatcaggttctacgaggaccaatcccatccgcccaaggccgagctgtcggcctgcgtcatcacccagggggcgatcctggcccaattgcaagccatccagaaatcccgccaagaattcttgctgaaaaagggccgcggggtctacctcgacccccagaccggtgaggagctcaaccccggcttcccccaggatgccccgaggaaacaagaagctgaaagtggagctgccgcccgtggaggatttggaggaagactgggagaacagcagtcaggcagaggaggaggagatggaggaagactgggacagcactcaggcagaggaggacagcctgcaagacagtctggaggaagacgaggaggaggcagaggaggaggtggaagaagcagccgccgccagaccgtcgtcctcggcgggggagaaagcaagcagcacggataccatctccgctccgggtcggggtcccgctcgaccacacagtagatgggacgagaccggacgattcccgaaccccaccacccagaccggtaagaaggagcggcagggatacaagtcctggcgggggcacaaaaacgccatcgtctcctgcttgcaggcctgcgggggcaacatctccttcacccggcgctacctgctcttccaccgcggggtgaactttccccgcaacatcttgcattactaccgtcacctccacagcccctactacttccaagaagaggcagcagcagcagaaaaagaccagcagaaaaccagcagctagaaaatccacagcggcggcagcaggtggactgaggatcgcggcgaacgagccggcgcaaacccgggagctgaggaaccggatctttcccaccctctatgccatcttccagcagagtcgggggcaggagcaggaactgaaagtcaagaaccgttctctgcgctcgctcacccgcagttgtctgtatcacaagagcgaagaccaacttcagcgcactctcgaggacgccgaggctctcttcaacaagtactgcgcgctcactcttaaagagtagcccgcgcccgcccagtcgcagaaaaaggcgggaattacgtcacctgtgcccttcgccctagccgcctccacccatcatcatgagcaaagagattcccacgccttacatgtggagctaccagccccagatgggcctggccgccggtgccgcccaggactactccacccgcatgaattggctcagcgccgggcccgcgatgatctcacgggtgaatgacatccgcgcccaccgaaaccagatactcctagaacagtcagcgctcaccgccacgccccgcaatcacctcaatccgcgtaattggcccgccgccctggtgtaccaggaaattccccagcccacgaccgtactacttccgcgagacgcccaggccgaagtccagctgactaactcaggtgtccagctggcgggcggcgccaccctgtgtcgtcaccgccccgctcagggtataaagcggctggtgatccggggcagaggcacacagctcaacgacgaggtggtgagctcttcgctgggtctgcgacctgacggagtcttccaactcgccggatcggggagatcttccttcacgcctcgtcaggccgtcctgactttggagagttcgtcctcgcagccccgctcgggtggcatcggcactctccagttcgtggaggagttcactccctcggtctacttcaaccccttctccggctcccccggccactacccggacgagttcatcccgaacttcgacgccatcagcgagtcggtggacggctacgattgaatgtcccatggtggcgcagctgacctagctcggcttcgacacctggaccactgccgccgcttccgctgcttcgctcgggatctcgccgagtttgcctactttgagctgcccgaggagcaccctcagggcccggcccacggagtgcggatcgtcgtcgaagggggcctcgactcccacctgcttcggatcttcagccagcgtccgatcctggtcgagcgcgagcaaggacagacccttctgactctgtactgcatctgcaaccaccccggcctgcatgaaagtctttgttgtctgctgtgtactgagtataataaaagctgagatcagcgactactccggacttccgtgtgttcctgaatccatcaaccagtctttgttcttcaccgggaacgagaccgagctccagctccagtgtaagccccacaagaagtacctcacctggctgttccagggctccccgatcgccgttgtcaaccactgcgacaacgacggagtcctgctgagcggccctgccaaccttactttttccacccgcagaagcaagctccagctcttccaacccttcctccccgggacctatcagtgcgtctcgggaccctgccatcacaccttccacctgatcccgaataccacagcgtcgctccccgctactaacaaccaaactaacctccaccaacgccaccgtcgctaggccacaatacatgcccatattagactatgaggccgagccacagcgacccatgctccccgctattagttacttcaatctaaccggcggagatgactgacccactggccaacaacaacgtcaacgaccttctcctggacatggacggccgcgcctcggagcagcgactcgcccaacttcgcattcgccagcagcaggagagagccgtcaaggagctgcaggatgcggtggccatccaccagtgcaagagaggcatcttctgcctggtgaaacaggccaagatctcctacgaggtcactccaaacgaccatcgcctctcctacgagctcctgcagcagcgccagaagttcacctgcctggtcggagtcaaccccatcgtcatcacccagcagtctggcgataccaaggggtgcatccactgctcctgcgactcccccgactgcgtccacactctgatcaagaccctctgcggcctccgcgacctcctccccatgaactaatcacccccttatccagtgaaataaagatcatattgatgatgattttacagaaataaaaaataatcatttgatttgaaataaagatacaatcatattgatgatttgagtttaacaaaaaaataaagaatcacttacttgaaatctgataccaggtctctgtccatgttttctgccaacaccacttcactcccctcttcccagctctggtactgcaggccccggcgggctgcaaacttcctccacacgctgaaggggatgtcaaattcctcctgtccctcaatcttcattttatcttctatcagatgtccaaaaagcgcgtccgggtggatgatgacttcgaccccgtctacccctacgatgcagacaacgcaccgaccgtgcccttcatcaacccccccttcgtctcttcagatggattccaagagaagcccctgggggtgttgtccctgcgactggccgaccccgtcaccaccaagaacggggaaatcaccctcaagctgggagagggggtggacctcgattcctcgggaaaactcatctccaacacggccaccaaggccgccgcccctctcagtttttccaacaacaccatttcccttaacatggatcaccccttttacactaaagatggaaaattatccttacaagtttctccaccattaaatatactgagaacaagcattctaaacacactagctttaggttttggatcaggtttaggactccgtggctctgccttggcagtacagttagtctctccacttacatttgatactgatggaaacataaagcttaccttagacagaggtttgcatgttacaacaggagatgcaattgaaagcaacataagctgggctaaaggtttaaaatttgaagatggagccatagcaaccaacattggaaatgggttagagtttggaagcagtagtacagaaacaggtgttgatgatgcttacccaatccaagttaaacttggatctggccttagctttgacagtacaggagccataatggctggtaacaaagaagacgataaactcactttgtggacaacacctgatccatcaccaaactgtcaaatactcgcagaaaatgatgcaaaactaacactttgcttgactaaatgtggtagtcaaatactggccactgtgtcagtcttagttgtaggaagtggaaacctaaaccccattactggcaccgtaagcagtgctcaggtgtttctacgttttgatgcaaacggtgttcttttaacagaacattctacactaaaaaaatactgggggtataggcagggagatagcatagatggcactccatataccaatgctgtaggattcatgcccaatttaaaagcttatccaaagtcacaaagttctactactaaaaataatatagtagggcaagtatacatgaatggagatgtttcaaaacctatgcttctcactataaccctcaatggtactgatgacagcaacagtacatattcaatgtcattttcatacacctggactaatggaagctatgttggagcaacatttggggctaactcttataccttctcatacatcgcccaagaatgaacactgtatcccaccctgcatgccaacccttcccaccccactctgtggaacaaactctgaaacacaaaataaaataaagttcaagtgttttattgattcaacagttttacaggattcgagcagttatttttcctccaccctcccaggacatggaatacaccaccctctccccccgcacagccttgaacatctgaatgccattggtgatggacatgcttttggtctccacgttccacacagtttcagagcgagccagtctcgggtcggtcagggagatgaaaccctccgggcactcccgcatctgcacctcacagctcaacagctgaggattgtcctcggtggtcgggatcacggttatctggaagaagcagaagagcggcggtgggaatcatagtccgcgaacgggatcggccggtggtgtcgcatcaggccccgcagcagtcgctgccgccgccgctccgtcaagctgctgctcagggggtccgggtccagggactccctcagcatgatgcccacggccctcagcatcagtcgtctggtgcggcgggcgcagcagcgcatgcggatctcgctcaggtcgctgcagtacgtgcaacacagaaccaccaggttgttcaacagtccatagttcaacacgctccagccgaaactcatcgcgggaaggatgctacccacgtggccgtcgtaccagatcctcaggtaaatcaagtggtgccccctccagaacacgctgcccacgtacatgatctccttgggcatgtggcggttcaccacctcccggtaccacatcaccctctggttgaacatgcagccccggatgatcctgcggaaccacagggccagcaccgccccgcccgccatgcagcgaagagaccccgggtcccggcaatggcaatggaggacccaccgctcgtacccgtggatcatctgggagctgaacaagtctatgttggcacagcacaggcatatgctcatgcatctcttcagcactctcaactcctcgggggtcaaaaccatatcccagggcacggggaactcttgcaggacagcgaaccccgcagaacagggcaatcctcgcacagaacttacattgtgcatggacagggtatcgcaatcaggcagcaccgggtgatcctccaccagagaagcgcgggtctcggtctcctcacagcgtggtaagggggccggccgatacgggtgatggcgggacgcggctgatcgtgttcgcgaccgtgtcatgatgcagttgctttcggacattttcgtacttgctgtagcagaacctggtccgggcgctgcacaccgatcgccggcggcggtctcggcgcttggaacgctcggtgttgaaattgtaaaacagccactctctcagaccgtgcagcagatctagggcctcaggagtgatgaagatcccatcatgcctgatggctctgatcacatcgaccaccgtggaatgggccagacccagccagatgatgcaattttgttgggtttcggtgacggcgggggagggaagaacaggaagaaccatgattaacttttaatccaaacggtctcggagtacttcaaaatgaagatcgcggagatggcacctctcgcccccgctgtgttggtggaaaataacagccaggtcaaaggtgatacggttctcgagatgttccacggtggcttccagcaaagcctccacgcgcacatccagaaacaagacaatagcgaaagcgggagggttctctaattcctcaatcatcatgttacactcctgcaccatccccagataattttcatttttccagccttgaatgattcgaactagttcctgaggtaaatccaagccagccatgataaagagctcgcgcagagcgccctccaccggcattcttaagcacaccctcataattccaagatattctgctcctggttcacctgcagcagattgacaagcggaatatcaaaatctctgccgcgatccctgagctcctccctcagcaataactgtaagtactctttcatatcctctccgaaatttttagccataggaccaccaggaataagattagggcaagccacagtacagataaaccgaagtcctccccagtgagcattgccaaatgcaagactgctataagcatgctggctagacccggtgatatcttccagataactggacagaaaatcgcccaggcaatttttaagaaaatcaacaaaagaaaaatcctccaggtggacgtttagagcctcgggaacaacgatgaagtaaatgcaagcggtgcgttccagcatggttagttagctgatctgtagaaaaaacaaaaatgaacattaaaccatgctagcctggcgaacaggtgggtaaatcgttctctccagcaccaggcaggccacggggtctccggcgcgaccctcgtaaaaattgtcgctatgattgaaaaccatcacagagagacgttcccggtggccggcgtgaatgattcgacaagatgaatacacccccggaacattggcgtccgcgagtgaaaaaaagcgcccgaggaagcaataaggcactacaatgctcagtctcaagtccagcaaagcgatgccatgcggatgaagcacaaaattctcaggtgcgtacaaaatgtaattactcccctcctgcacaggcagcaaagcccccgatccctccaggtacacatacaaagcctcagcgtccatagcttaccgagcagcagcacacaacaggcgcaagagtcagagaaaggctgagctctaacctgtccacccgctctctgctcaatatatagcccagatctacactgacgtaaaggccaaagtctaaaaatacccgccaaataatcacacacgcccagcacacgcccagaaaccggtgacacactcaaaaaaatacgcgcacttcctcaaacgcccaaaactgccgtcatttccgggttcccacgctacgtcatcaaaacacgactttcaaattccgtcgaccgttaaaaacgtcacccgccccgcccctaacggtcgcccgtctctcagccaatcagcgccccgcatccccaaattcaaacacctcatttgcatattaacgcgcacaaaaagtttgaggtatattattgatgatgg

SEQ ID NO: 46 - DNA, 7182 bp, synthetic construct
  misc_feature 1..7182: note = Synthetic Construct
  source 1..7182: mol_type = other DNA
ggcgtaatgctctgccagtgttacaaccaattaaccaattctgattagaaaaactcatcgagcatcaaatgaaactgcaatttattcatatcaggattatcaataccatatttttgaaaaagccgtttctgtaatgaaggagaaaactcaccgaggcagttccataggatggcaagatcctggtatcggtctgcgattccgactcgtccaacatcaatacaacctattaatttcccctcgtcaaaaataaggttatcaagtgagaaatcaccatgagtgacgactgaatccggtgagaatggcaaaagcttatgcatttctttccagacttgttcaacaggccagccattacgctcgtcatcaaaatcactcgcatcaaccaaaccgttattcattcgtgattgcgcctgagcgagacgaaatacgcgatcgctgttaaaaggacaattacaaacaggaatcaaatgcaaccggcgcaggaacactgccagcgcatcaacaatattttcacctgaatcaggatattcttctaatacctggaatgctgttttcccggggatcgcagtggtgagtaaccatgcatcatcaggagtacggataaaatgcttgatggtcggaagaggcataaattccgtcagccagtttagtctgaccatctcatctgtaacatcattggcaacgctacctttgccatgtttcagaaacaactctggcgcatcgggcttcccatacaatcgatagattgtcgcacctgattgcccgacattatcgcgagcccatttatacccatataaatcagcatccatgttggaatttaatcgcggcctcgagcaagacgtttcccgttgaatatggctcataacaccccttgtattactgtttatgtaagcagacaggtcgacaatattggctattggccattgcatacgttgtatctatatcataatatgtacatttatattggctcatgtccaatatgaccgccatgttgacattgattattgactagttattaatagtaatcaattacggggtcattagttcatagcccatatatggagttccgcgttacataacttacggtaaatggcccgcctggctgaccgcccaacgacccccgcccattgacgtcaataatgacgtatgttcccatagtaacgccaatagggactttccattgacgtcaatgggtggagtatttacggtaaactgcccacttggcagtacatcaagtgtatcatatgccaagtccgccccctattgacgtcaatgacggtaaatggcccgcctggcattatgcccagtacatgaccttacgggactttcctacttggcagtacatctacgtattagtcatcgctattaccatggtgatgcggttttggcagtacaccaatgggcgtggatagcggtttgactcacggggatttccaagtctccaccccattgacgtcaatgggagtttgttttggcaccaaaatcaacgggactttccaaaatgtcgtaataaccccgccccgttgacgcaaatgggcggtaggcgtgtacggtgggaggtctatataagcagagctcgtttagtgaaccgtcagatcgcctggagacgccatccacgctgttttgacctccatagaagacaccgggaccgatccagcctccgcggccgggaacggtgcattggaacgcggattccccgtgccaagagtgactcaccgtccggatctcagcaagcaggtatgtactctccagggtgggcctggcttccccagtcaagactccagggatttgagggacgctgtgggctcttctcttacatgtaccttttgcttgcctcaaccctgactatcttccaggtcaggatcccagagtcaggggtctgtattttcctgctggtggctccagttcaggaacagtaaaccctgctccgaatattgcctctcacatctcgtcaatctccgcgaggactggggaccctgtgacgaacatggctagcattgtgggaggctgggagtgcgagaagcattcccaaccctggcaggtgcttgtggcctctcgtggcagggcagtctgcggcggtgttctggtgcacccccagtgggtcctcacagctgcccactgcatcaggaacaaaagcgtgatcttgctgggtcggcacagcttgtttcatcctgaagacacaggccaggtatttcaggtcagccacagcttcccacacccgctctacgatatgagcctcctgaagaatcgattcctcaggccaggtgatgactccagccacgacctcatgctgctccgcctgtcagagcctgccgagctcacggatgctgtgaaggtcatggacctgcccacccaggagccagcactggggaccacctgctacgcctcaggctggggcagcattgaaccagaggagttcttgaccccaaagaaacttcagtgtgtggacctccatgttatttccaatgacgtgtgtgcgcaagttcaccctcagaaggtgaccaagttcatgctgtgtgctggacgctggacagggggcaaaagcacctgctcgggtgattctgggggcccacttgtctgtaatggtgtgcttcaaggtatcacgtcatggggcagtgaaccatgtgccctgcccgaaaggccttccctgtacaccaaggtggtgcattaccggaagtggatcaaggacaccatcgtggccaaccccggatccgaaggtaggggttcattattgacctgtggagatgtcgaagaaaacccaggacccgctagcaaggctgtgctgcttgccctgttgatggcaggcttggccctgcagccaggcactgccctgctgtgctactcctgcaaagcccaggtgagcaacgaggactgcctgcaggtggagaactgcacccagctgggggagcagtgctggaccgcgcgcatccgcgcagttggcctcctgaccgtcatcagcaaaggctgcagcttgaactgcgtggatgactcacaggactactacgtgggcaagaagaacatcacgtgctgtgacaccgacttgtgcaacgccagcggggcccatgccctgcagccggctgccgccatccttgcgctgctccctgcactcggcctgctgctctggggacccggccagctaggatcccagaccctgaactttgatctgctgaaactggcaggcgatgtggaaagcaacccaggcccaatggcaagcgcgcgccgcccgcgctggctgtgcgctggggcgctggtgctggcgggtggcttctttctcctcggcttcctcttcgggtggtttataaaatcctccaatgaagctactaacattactccaaagcataatatgaaagcatttttggatgaattgaaagctgagaacatcaagaagttcttatataattttacacagataccacatttagcaggaacagaacaaaactttcagcttgcaaagcaaattcaatcccagtggaaagaatttggcctggattctgttgagctggcacattatgatgtcctgttgtcctacccaaataagactcatcccaactacatctcaataattaatgaagatggaaatgagattttcaacacatcattatttgaaccacctcctccaggatatgaaaatgtttcggatattgtaccacctttcagtgctttctctcctcaaggaatgccagagggcgatctagtgtatgttaactatgcacgaactgaagacttctttaaattggaacgggacatgaaaatcaattgctctgggaaaattgtaattgccagatatgggaaagttttcagaggaaataaggttaaaaatgcccagctggcaggggccaaaggagtcattctctactccgaccctgctgactactttgctcctggggtgaagtcctatccagatggttggaatcttcctggaggtggtgtccagcgtggaaatatcctaaatctgaatggtgcaggagaccctctcacaccaggttacccagcaaatgaatatgcttataggcgtggaattgcagaggctgttggtcttccaagtattcctgttcatccaattggatactatgatgcacagaagctcctagaaaaaatgggtggctcagcaccaccagatagcagctggagaggaagtctcaaagtgccctacaatgttggacctggctttactggaaacttttctacacaaaaagtcaagatgcacatccactctaccaatgaagtgacaagaatttacaatgtgataggtactctcagaggagcagtggaaccagacagatatgtcattctgggaggtcaccgggactcatgggtgtttggtggtattgaccctcagagtggagcagctgttgttcatgaaattgtgaggagctttggaacactgaaaaaggaagggtggagacctagaagaacaattttgtttgcaagctgggatgcagaagaatttggtcttcttggttctactgagtgggcagaggagaattcaagactccttcaagagcgtggcgtggcttatattaatgctgactcatctatagaaggaaactacactctgagagttgattgtacaccgctgatgtacagcttggtacacaacctaacaaaagagctgaaaagccctgatgaaggctttgaaggcaaatctctttatgaaagttggactaaaaaaagtccttccccagagttcagtggcatgcccaggataagcaaattgggatctggaaatgattttgaggtgttcttccaacgacttggaattgcttcaggcagagcacggtatactaaaaattgggaaacaaacaaattcagcggctatccactgtatcacagtgtctatgaaacatatgagttggtggaaaagttttatgatccaatgtttaaatatcacctcactgtggcccaggttcgaggagggatggtgtttgagctggccaattccatagtgctcccttttgattgtcgagattatgctgtagttttaagaaagtatgctgacaaaatctacagtatttctatgaaacatccacaggaaatgaagacatacagtgtatcatttgattcacttttttctgcagtaaagaattttacagaaattgcttccaagttcagtgagagactccaggactttgacaaaagcaacccaatagtattaagaatgatgaatgatcaactcatgtttctggaaagagcatttattgatccattagggttaccagacaggcctttttataggcatgtcatctatgctccaagcagccacaacaagtatgcaggggagtcattcccaggaatttatgatgctctgtttgatattgaaagcaaagtggacccttccaaggcctggggagaagtgaagagacagatttatgttgcagccttcacagtgcaggcagctgcagagactttgagtgaagtagcctaaagatctgggccctaacaaaacaaaaagatggggttattccctaaacttcatgggttacgtaattggaagttgggggacattgccacaagatcatattgtacaaaagatcaaacactgttttagaaaacttcctgtaaacaggcctattgattggaaagtatgtcaaaggattgtgggtcttttgggctttgctgctccatttacacaatgtggatatcctgccttaatgcctttgtatgcatgtatacaagctaaacaggctttcactttctcgccaacttacaaggcctttctaagtaaacagtacatgaacctttaccccgttgctcggcaacggcctggtctgtgccaagtgtttgctgacgcaacccccactggctggggcttggccataggccatcagcgcatgcgtggaacctttgtggctcctctgccgatccatactgcggaactcctagccgcttgttttgctcgcagccggtctggagcaaagctcataggaactgacaattctgtcgtcctctcgcggaaatatacatcgtttcgatctacgtatgatctttttccctctgccaaaaattatggggacatcatgaagccccttgagcatctgacttctggctaataaaggaaatttattttcattgcaatagtgtgttggaattttttgtgtctctcactcggaaggaattctgcattaatgaatcggccaacgcgcggggagaggcggtttgcgtattgggcgctcttccgcttcctcgctcactgactcgctgcgctcggtcgttcggctgcggcgagcggtatcagctcactcaaaggcggtaatacggttatccacagaatcaggggataacgcaggaaagaacatgtgagcaaaaggccagcaaaaggccaggaaccgtaaaaaggccgcgttgctggcgtttttccataggctccgcccccctgacgagcatcacaaaaatcgacgctcaagtcagaggtggcgaaacccgacaggactataaagataccaggcgtttccccctggaagctccctcgtgcgctctcctgttccgaccctgccgcttaccggatacctgtccgcctttctcccttcgggaagcgtggcgctttctcatagctcacgctgtaggtatctcagttcggtgtaggtcgttcgctccaagctgggctgtgtgcacgaaccccccgttcagcccgaccgctgcgccttatccggtaactatcgtcttgagtccaacccggtaagacacgacttatcgccactggcagcagccactggtaacaggattagcagagcgaggtatgtaggcggtgctacagagttcttgaagtggtggcctaactacggctacactagaagaacagtatttggtatctgcgctctgctgaagccagttaccttcggaaaaagagttggtagctcttgatccggcaaacaaaccaccgctggtagcggtggtttttttgtttgcaagcagcagattacgcgcagaaaaaaaggatctcaagaagatcctttgatcttttctacggggtctgacgctcagtggaacgaaaactcacgttaagggattttggtcatgagattatcaaaaaggatcttcacctagatccttttaaattaaaaatgaagttttaaatcaatctaaagtatatatgagtaaacttggtctgacagttaccaatgcttaatcagtgaggcacctatctcagcgatctgtctatttcgttcatccatagttgcctgactc

SEQ ID NO: 47 - protein, 261 aa, Homo sapiens
MWVPVVFLTLSVTWIGAAPLILSRIVGGWECEKHSQPWQVLVASRGRAVCGGVLVHPQWVLTAAHCIRNKSVILLGRHSLFHPEDTGQVFQVSHSFPHPLYDMSLLKNRFLRPGDDSSHDLMLLRLSEPAELTDAVKVMDLPTQEPALGTTCYASGWGSIEPEEFLTPKKLQCVDLHVISNDVCAQVHPQKVTKFMLCAGRWTGGKSTCSGDSGGPLVCNGVLQGITSWGSEPCALPERPSLYTKVVHYRKWIKDTIVANP

SEQ ID NO: 48 - protein, 123 aa, Homo sapiens
MKAVLLALLMAGLALQPGTALLCYSCKAQVSNEDCLQVENCTQLGEQCWTARIRAVGLLTVISKGCSLNCVDDSQDYYVGKKNITCCDTDLCNASGAHALQPAAAILALLPALGLLLWGPGQL

SEQ ID NO: 49 - DNA, 24 bp, synthetic construct
  misc_feature 1..24: note = Synthetic Construct
  source 1..24: mol_type = other DNA
tcgtcgttttgtcgttttgtcgtt

SEQ ID NO: 50 - DNA, 21 bp, synthetic construct
  misc_feature 1..21: note = Synthetic Construct
  source 1..21: mol_type = other DNA
tcgtcgtttttcggtgctttt

SEQ ID NO: 51 - DNA, 21 bp, synthetic construct
  misc_feature 1..21: note = Synthetic Construct
  source 1..21: mol_type = other DNA
tcgtcgtttttcggtcgtttt